European Patent Application EP 4 317 185 A2, published February 7, 2024. Title: FULLY-HUMAN POST-TRANSLATIONALLY MODIFIED ANTIBODY THERAPEUTICS. Applicant: REGENXBIO Inc. Application EP. The sequence listing filed with the application follows.

SEQUENCE LISTING (314 sequences)

SEQ ID NO: 1 - protein, 249 aa, synthetic construct
  MOD_RES 1: note = Any amino acid
  SITE 229..249: note = /note="This region may be absent in its entirety"
  VARIANT 232: note = L
  SITE 233..249: note = /note="This region may be absent in its entirety"
  SITE 239..249: note = /note="This region may be absent in its entirety"
  SITE 1..249: note = /note="Variant residues given in the sequence have no preference with respect to those in the annotations for variant positions"
  REGION 1..249: note = source = /note="Description of Artificial Sequence: Synthetic polypeptide"
  REGION 1..249: note = source = /note="See specification as filed for detailed description of substitutions and preferred embodiments"
XVQLVESGGGVVQPGRSLRLSCAASGFAFSSYGMHWVRQAPGKGLEWVAVIWFDGTKKYYTDSVKGRFTISRDNSKNTLYLQMNTLRAEDTAVYYCARDRGIGARRGPYYMDVWGKGTTVTVSSASTKGPSVFPLAPSSKSTSGGTAALGCLVKDYFPEPVTVSWNSGALTSGVHTFPAVLQSSGLYSLSSVVTVPSSSLGTQTYICNVNHKPSNTKVDKRVEPKSCDKTHTCPPCPAPELLGGPSVFL

SEQ ID NO: 2 - protein, 214 aa, synthetic construct
  REGION 1..214: note = source = /note="Description of Artificial Sequence: Synthetic polypeptide"
DIQMTQSPSSLSASVGDRVTITCRASQSISSYLNWYQQKPGKAPKLLIYAASSLQSGVPSRFSGSGSGTDFTLTISSLQPEDFATYYCQQSYSTPLTFGGGTKVEIKRTVAAPSVFIFPPSDEQLKSGTASVVCLLNNFYPREAKVQWKVDNALQSGNSQESVTEQDSKDSTYSLSSTLTLSKADYEKHKVYACEVTHQGLSSPVTKSFNRGEC

SEQ ID NO: 3 - protein, 234 aa, synthetic construct
  SITE 215..234: note = /note="This region may be absent in its entirety"
  SITE 224..234: note = /note="This region may be absent in its entirety"
  SITE 1..234: note = /note="Variant residues given in the sequence have no preference with respect to those in the annotations for variant positions"
  REGION 1..234: note = source = /note="Description of Artificial Sequence: Synthetic polypeptide"
  REGION 1..234: note = source = /note="See specification as filed for detailed description of substitutions and preferred embodiments"
EVQLVESGGGLVQPGGSLRLSCAASGFTFSSYGMSWVRQAPGKGLELVASINSNGGSTYYPDSVKGRFTISRDNAKNSLYLQMNSLRAEDTAVYYCASGDYWGQGTTVTVSSASTKGPSVFPLAPCSRSTSESTAALGCLVKDYFPEPVTVSWNSGALTSGVHTFPAVLQSSGLYSLSSVVTVPSSSLGTKTYTCNVDHKPSNTKVDKRVESKYGPPCPPCPAPEFLGGPSVFL

SEQ ID NO: 4 - protein, 219 aa, synthetic construct
  REGION 1..219: note = source = /note="Description of Artificial Sequence: Synthetic polypeptide"
DIVMTQSPLSLPVTPGEPASISCRSSQSLVYSNGDTYLHWYLQKPGQSPQLLIYKVSNRFSGVPDRFSGSGSGTDFTLKISRVEAEDVGVYYCSQSTHVPWTFGQGTKVEIKRTVAAPSVFIFPPSDEQLKSGTASVVCLLNNFYPREAKVQWKVDNALQSGNSQESVTEQDSKDSTYSLSSTLTLSKADYEKHKVYACEVTHQGLSSPVTKSFNRGEC

SEQ ID NO: 5 - protein, 251 aa, synthetic construct
  SITE 231..251: note = /note="This region may be absent in its entirety"
  VARIANT 234: note = L
  SITE 235..251: note = /note="This region may be absent in its entirety"
  SITE 241..251: note = /note="This region may be absent in its entirety"
  SITE 1..251: note = /note="Variant residues given in the sequence have no preference with respect to those in the annotations for variant positions"
  REGION 1..251: note = source = /note="Description of Artificial Sequence: Synthetic polypeptide"
  REGION 1..251: note = source = /note="See specification as filed for detailed description of substitutions and preferred embodiments"
QVELVESGGGLVQPGGSLRLSCAASGFTFSSYAMSWVRQAPGKGLEWVSAINASGTRTYYADSVKGRFTISRDNSKNTLYLQMNSLRAEDTAVYYCARGKGNTHKPYGYVRYFDVWGQGTLVTVSSASTKGPSVFPLAPSSKSTSGGTAALGCLVKDYFPEPVTVSWNSGALTSGVHTFPAVLQSSGLYSLSSVVTVPSSSLGTQTYICNVNHKPSNTKVDKKVEPKSCDKTHTCPPCPAPELLGGPSVFL

SEQ ID NO: 6 - protein, 215 aa, synthetic construct
  REGION 1..215: note = source = /note="Description of Artificial Sequence: Synthetic polypeptide"
DIVLTQSPATLSLSPGERATLSCRASQSVSSSYLAWYQQKPGQAPRLLIYGASSRATGVPARFSGSGSGTDFTLTISSLEPEDFATYYCLQIYNMPITFGQGTKVEIKRTVAAPSVFIFPPSDEQLKSGTASVVCLLNNFYPREAKVQWKVDNALQSGNSQESVTEQDSKDSTYSLSSTLTLSKADYEKHKVYACEVTHQGLSSPVTKSFNRGEC

SEQ ID NO: 7 - protein, 247 aa, synthetic construct
  SITE 228..247: note = /note="This region may be absent in its entirety"
  SITE 237..247: note = /note="This region may be absent in its entirety"
  SITE 1..247: note = /note="Variant residues given in the sequence have no preference with respect to those in the annotations for variant positions"
  REGION 1..247: note = source = /note="Description of Artificial Sequence: Synthetic polypeptide"
  REGION 1..247: note = source = /note="See specification as filed for detailed description of substitutions and preferred embodiments"
EVQLVESGGGLEQPGGSLRLSCAGSGFTFRDYAMTWVRQAPGKGLEWVSSISGSGGNTYYADSVKGRFTISRDNSKNTLYLQMNSLRAEDTAVYYCAKDRLSITIRPRYYGLDVWGQGTTVTVSSASTKGPSVFPLAPCSRSTSESTAALGCLVKDYFPEPVTVSWNSGALTSGVHTFPAVLQSSGLYSLSSVVTVPSSSLGTKTYTCNVDHKPSNTKVDKRVESKYGPPCPPCPAPEFLGGPSVFL

SEQ ID NO: 8 - protein, 219 aa, synthetic construct
  REGION 1..219: note = source = /note="Description of Artificial Sequence: Synthetic polypeptide"
DIVMTQSPLSLPVTPGEPASISCRSSQSLLYSIGYNYLDWYLQKSGQSPQLLIYLGSNRASGVPDRFSGSGSGTDFTLKISRVEAEDVGFYYCMQALQTPYTFGQGTKLEIKRTVAAPSVFIFPPSDEQLKSGTASVVCLLNNFYPREAKVQWKVDNALQSGNSQESVTEQDSKDSTYSLSSTLTLSKADYEKHKVYACEVTHQGLSSPVTKSFNRGEC

SEQ ID NO: 9 - protein, 241 aa, synthetic construct
  SITE 222..241: note = /note="This region may be absent in its entirety"
  SITE 231..241: note = /note="This region may be absent in its entirety"
  SITE 1..241: note = /note="Variant residues given in the sequence have no preference with respect to those in the annotations for variant positions"
  REGION 1..241: note = source = /note="Description of Artificial Sequence: Synthetic polypeptide"
  REGION 1..241: note = source = /note="See specification as filed for detailed description of substitutions and preferred embodiments"
QVQLVQSGAEVKKPGSSVKVSCKASGYSFTDYHIHWVRQAPGQGLEWMGVINPMYGTTDYNQRFKGRVTITADESTSTAYMELSSLRSEDTAVYYCARYDYFTGTGVYWGQGTLVTVSSASTKGPSVFPLAPCSRSTSESTAALGCLVKDYFPEPVTVSWNSGALTSGVHTFPAVLQSSGLYSLSSVVTVPSSSLGTKTYTCNVDHKPSNTKVDKRVESKYGPPCPPCPAPEFLGGPSVFL

SEQ ID NO: 10 - protein, 219 aa, synthetic construct
  REGION 1..219: note = source = /note="Description of Artificial Sequence: Synthetic polypeptide"
DIVMTQTPLSLSVTPGQPASISCRSSRSLVHSRGNTYLHWYLQKPGQSPQLLIYKVSNRFIGVPDRFSGSGSGTDFTLKISRVEAEDVGVYYCSQSTHLPFTFGQGTKLEIKRTVAAPSVFIFPPSDEQLKSGTASVVCLLNNFYPREAKVQWKVDNALQSGNSQESVTEQDSKDSTYSLSSTLTLSKADYEKHKVYACEVTHQGLSSPVTKSFNRGEC

SEQ ID NO: 11 - protein, 252 aa, synthetic construct
  SITE 232..252: note = /note="This region may be absent in its entirety"
  VARIANT 235: note = L
  SITE 236..252: note = /note="This region may be absent in its entirety"
  SITE 242..252: note = /note="This region may be absent in its entirety"
  SITE 1..252: note = /note="Variant residues given in the sequence have no preference with respect to those in the annotations for variant positions"
  REGION 1..252: note = source = /note="Description of Artificial Sequence: Synthetic polypeptide"
  REGION 1..252: note = source = /note="See specification as filed for detailed description of substitutions and preferred embodiments"
EVQLVESGGGLVQPGGSLRLSCAASGFTFSNYWMNWVRQAPGKGLEWVAAINQDGSEKYYVGSVKGRFTISRDNAKNSLYLQMNSLRVEDTAVYYCVRDYYDILTDYYIHYWYFDLWGRGTLVTVSSASTKGPSVFPLAPSSKSTSGGTAALGCLVKDYFPEPVTVSWNSGALTSGVHTFPAVLQSSGLYSLSSVVTVPSSSLGTQTYICNVNHKPSNTKVDKRVEPKSCDKTHTCPPCPAPELLGGPSVFL

SEQ ID NO: 12 - protein, 215 aa, synthetic construct
  REGION 1..215: note = source = /note="Description of Artificial Sequence: Synthetic polypeptide"
EIVLTQSPGTLSLSPGERATLSCRASQSVSSSYLAWYQQKPGQAPRLLIYGASSRATGIPDRFSGSGSGTDFTLTISRLEPEDFAVYYCQQYGSSPCTFGQGTRLEIKRTVAAPSVFIFPPSDEQLKSGTASVVCLLNNFYPREAKVQWKVDNALQSGNSQESVTEQDSKDSTYSLSSTLTLSKADYEKHKVYACEVTHQGLSSPVTKSFNRGEC

SEQ ID NO: 13 - protein, 244 aa, synthetic construct
  SITE 224..244: note = /note="This region may be absent in its entirety"
  VARIANT 227: note = L
  SITE 228..244: note = /note="This region may be absent in its entirety"
  SITE 234..244: note = /note="This region may be absent in its entirety"
  SITE 1..244: note = /note="Variant residues given in the sequence have no preference with respect to those in the annotations for variant positions"
  REGION 1..244: note = source = /note="Description of Artificial Sequence: Synthetic polypeptide"
  REGION 1..244: note = source = /note="See specification as filed for detailed description of substitutions and preferred embodiments"
EVQLVQSGAEVKKPGESLKISCKGSGYSFTTYWLGWVRQMPGKGLDWIGIMSPVDSDIRYSPSFQGQVTMSVDKSITTAYLQWNSLKASDTAMYYCARRRPGQGYFDFWGQGTLVTVSSSSTKGPSVFPLAPSSKSTSGGTAALGCLVKDYFPEPVTVSWNSGALTSGVHTFPAVLQSSGLYSLSSVVTVPSSSLGTQTYICNVNHKPSNTKVDKRVEPKSCDKTHTCPPCPAPELLGGPSVFL

SEQ ID NO: 14 - protein, 214 aa, synthetic construct
  REGION 1..214: note = source = /note="Description of Artificial Sequence: Synthetic polypeptide"
DIQMTQSPSSLSASVGDRVTITCRASQGISSWLAWYQQKPEKAPKSLIYAASSLQSGVPSRFSGSGSGTDFTLTISSLQPEDFATYYCQQYNIYPYTFGQGTKLEIKRTVAAPSVFIFPPSDEQLKSGTASVVCLLNNFYPREAKVQWKVDNALQSGNSQESVTEQDSKDSTYSLSSTLTLSKADYEKHKVYACEVTHQGLSSPVTKSFNRGEC

SEQ ID NO: 15 - protein, 244 aa, synthetic construct
  SITE 224..244: note = /note="This region may be absent in its entirety"
  VARIANT 227: note = L
  SITE 228..244: note = /note="This region may be absent in its entirety"
  SITE 234..244: note = /note="This region may be absent in its entirety"
  SITE 1..244: note = /note="Variant residues given in the sequence have no preference with respect to those in the annotations for variant positions"
  REGION 1..244: note = source = /note="Description of Artificial Sequence: Synthetic polypeptide"
  REGION 1..244: note = source = /note="See specification as filed for detailed description of substitutions and preferred embodiments"
QVTLRESGPALVKPTQTLTLTCTVSGFSLTSYSVHWVRQPPGKGLEWLGVIWASGGTDYNSALMSRLSISKDTSRNQVVLTMTNMDPVDTATYYCARDPPSSLLRLDYWGRGTPVTVSSASTKGPSVFPLAPSSKSTSGGTAALGCLVKDYFPEPVTVSWNSGALTSGVHTFPAVLQSSGLYSLSSVVTVPSSSLGTQTYICNVNHKPSNTKVDKRVEPKSCDKTHTCPPCPAPELLGGPSVFL

SEQ ID NO: 16 - protein, 220 aa, synthetic construct
  MOD_RES 42: note = Any amino acid
  REGION 1..220: note = source = /note="Description of Artificial Sequence: Synthetic polypeptide"
DIVMTQSPDSLAVSLGERATINCKSSQSLLNSGNQKNYLAWXQQKPGQPPKLLIYGASTRESGVPDRFSGSGSGTDFTLTISSLQAEDVAVYYCQNVHSFPFTFGGGTKLEIKRTVAAPSVFIFPPSDEQLKSGTASVVCLLNNFYPREAKVQWKVDNALQSGNSQESVTEQDSKDSTYSLSSTLTLSKADYEKHKVYACEVTHQGLSSPVTKSFNRGEC

SEQ ID NO: 17 - protein, 246 aa, synthetic construct
  SITE 226..246: note = /note="This region may be absent in its entirety"
  VARIANT 229: note = L
  SITE 230..246: note = /note="This region may be absent in its entirety"
  SITE 236..246: note = /note="This region may be absent in its entirety"
  SITE 1..246: note = /note="Variant residues given in the sequence have no preference with respect to those in the annotations for variant positions"
  REGION 1..246: note = source = /note="Description of Artificial Sequence: Synthetic polypeptide"
  REGION 1..246: note = source = /note="See specification as filed for detailed description of substitutions and preferred embodiments"
QVQLVQSGAEVKKPGASVKVSCKGSGYTFTSYWMHWVRQAPGQRLEWIGEIDPSESNTNYNQKFKGRVTLTVDISASTAYMELSSLRSEDTAVYYCARGGYDGWDYAIDYWGQGTLVTVSSASTKGPSVFPLAPSSKSTSGGTAALGCLVKDYFPEPVTVSWNSGALTSGVHTFPAVLQSSGLYSLSSVVTVPSSSLGTQTYICNVNHKPSNTKVDKKVEPKSCDKTHTCPPCPAPELAGAPSVFL

SEQ ID NO: 18 - protein, 219 aa, synthetic construct
  REGION 1..219: note = source = /note="Description of Artificial Sequence: Synthetic polypeptide"
DVVMTQSPLSLPVTPGEPASISCRSSQSLAKSYGNTYLSWYLQKPGQSPQLLIYGISNRFSGVPDRFSGSGSGTDFTLKISRVEAEDVGVYYCLQGTHQPYTFGQGTKVEIKRTVAAPSVFIFPPSDEQLKSGTASVVCLLNNFYPREAKVQWKVDNALQSGNSQESVTEQDSKDSTYSLSSTLTLSKADYEKHKVYACEVTHQGLSSPVTKSFNRGEC

SEQ ID NO: 19 - protein, 245 aa, synthetic construct
  SITE 226..245: note = /note="This region may be absent in its entirety"
  SITE 235..245: note = /note="This region may be absent in its entirety"
  SITE 1..245: note = /note="Variant residues given in the sequence have no preference with respect to those in the annotations for variant positions"
  REGION 1..245: note = source = /note="Description of Artificial Sequence: Synthetic polypeptide"
  REGION 1..245: note = source = /note="See specification as filed for detailed description of substitutions and preferred embodiments"
QVQLVQSGAEVKKPGASVKVSCKASGFNIKDTYIHWVRQAPGQRLEWMGRIDPANGYTKYDPKFQGRVTITADTSASTAYMELSSLRSEDTAVYYCAREGYYGNYGVYAMDYWGQGTLVTVSSASTKGPSVFPLAPCSRSTSESTAALGCLVKDYFPEPVTVSWNSGALTSGVHTFPAVLQSSGLYSLSSVVTVPSSSLGTKTYTCNVDHKPSNTKVDKRVESKYGPPCPPCPAPEFLGGPSVFL

SEQ ID NO: 20 - protein, 213 aa, synthetic construct
  REGION 1..213: note = source = /note="Description of Artificial Sequence: Synthetic polypeptide"
DIQMTQSPSSLSASVGDRVTITCKTSQDINKYMAWYQQTPGKAPRLLIHYTSALQPGIPSRFSGSGSGRDYTFTISSLQPEDIATYYCLQYDNLWTFGQGTKVEIKRTVAAPSVFIFPPSDEQLKSGTASVVCLLNNFYPREAKVQWKVDNALQSGNSQESVTEQDSKDSTYSLSSTLTLSKADYEKHKVYACEVTHQGLSSPVTKSFNRGEC

SEQ ID NO: 21 - protein, 243 aa, synthetic construct
  SITE 223..243: note = /note="This region may be absent in its entirety"
  VARIANT 226: note = L
  SITE 227..243: note = /note="This region may be absent in its entirety"
  SITE 233..243: note = /note="This region may be absent in its entirety"
  SITE 1..243: note = /note="Variant residues given in the sequence have no preference with respect to those in the annotations for variant positions"
  REGION 1..243: note = source = /note="Description of Artificial Sequence: Synthetic polypeptide"
  REGION 1..243: note = source = /note="See specification as filed for detailed description of substitutions and preferred embodiments"
EVQLVESGGGLVQPGGSLRLSCAASGFTFNNYAMNWVRQAPGKGLDWVSTISGSGGTTNYADSVKGRFIISRDSSKHTLYLQMNSLRAEDTAVYYCAKDSNWGNFDLWGRGTLVTVSSASTKGPSVFPLAPSSKSTSGGTAALGCLVKDYFPEPVTVSWNSGALTSGVHTFPAVLQSSGLYSLSSVVTVPSSSLGTQTYICNVNHKPSNTKVDKKVEPKSCDKTHTCPPCPAPELLGGPSVFL

SEQ ID NO: 22 - protein, 220 aa, synthetic construct
  REGION 1..220: note = source = /note="Description of Artificial Sequence: Synthetic polypeptide"
DIVMTQSPDSLAVSLGERATINCKSSQSVLYRSNNRNFLGWYQQKPGQPPNLLIYWASTRESGVPDRFSGSGSGTDFTLTISSLQAEDVAVYYCQQYYTTPYTFGQGTKLEIKRTVAAPSVFIFPPSDEQLKSGTASVVCLLNNFYPREAKVQWKVDNALQSGNSQESVTEQDSKDSTYSLSSTLTLSKADYEKHKVYACEVTHQGLSSPVTKSFNRGEC

SEQ ID NO: 23 - protein, 231 aa, synthetic construct
  SITE 221..231: note = /note="This region may be absent in its entirety"
  SITE 227..231: note = /note="This region may be absent in its entirety"
  SITE 1..231: note = /note="Variant residues given in the sequence have no preference with respect to those in the annotations for variant positions"
  REGION 1..231: note = source = /note="Description of Artificial Sequence: Synthetic polypeptide"
  REGION 1..231: note = source = /note="See specification as filed for detailed description of substitutions and preferred embodiments"
EVQLVQSGAEVKKPGASVKVSCKASGYTLTSYGISWVRQAPGQGLEWMGWVSFYNGNTNYAQKLQGRGTMTTDPSTSTAYMELRSLRSDDTAVYYCARGYGMDVWGQGTTVTVSSASTKGPSVFPLAPCSRSTSESTAALGCLVKDYFPEPVTVSWNSGALTSGVHTFPAVLQSSGLYSLSSVVTVPSSNFGTQTYTCNVDHKPSNTKVDKTVERKCCVECPPCPAPPVAG

SEQ ID NO: 24 - protein, 215 aa, synthetic construct
  REGION 1..215: note = source = /note="Description of Artificial Sequence: Synthetic polypeptide"
ESALTQPASVSGSPGQSITISCTGTSSDVGGYNSVSWYQQHPGKAPKLMIYEVSNRPSGVSNRFSGSKSGNTASLTISGLQAEDEADYYCNSYTSTSMVFGGGTKLTVLGQPKAAPSVTLFPPSSEELQANKATLVCLISDFYPGAVTVAWKADSSPVKAGVETTTPSKQSNNKYAASSYLSLTPEQWKSHRSYSCQVTHEGSTVEKTVAPTECS

SEQ ID NO: 25 - protein, 248 aa, synthetic construct
  SITE 232..248: note = /note="This region may be absent in its entirety"
  SITE 238..248: note = /note="This region may be absent in its entirety"
  SITE 1..248: note = /note="Variant residues given in the sequence have no preference with respect to those in the annotations for variant positions"
  REGION 1..248: note = source = /note="Description of Artificial Sequence: Synthetic polypeptide"
  REGION 1..248: note = source = /note="See specification as filed for detailed description of substitutions and preferred embodiments"
EVQLVESGGGVIQPGGSLRLSCAASGFTFDDYAMNWVRQGPGKGLEWVSAISGDGGSTYYADSVKGRFTISRDNSKNSLYLQMNSLRAEDTAFFYCAKDLRNTIFGVVIPDAFDIWGQGTMVTVSSASTKGPSVFPLAPCSRSTSESTAALGCLVKDYFPEPVTVSWNSGALTSGVHTFPAVLQSSGLYSLSSVVTVPSSSLGTKTYTCNVDHKPSNTKVDKRVESKYGPPCPPCPAPEFLGGPSVFL

SEQ ID NO: 26 - protein, 214 aa, synthetic construct
  REGION 1..214: note = source = /note="Description of Artificial Sequence: Synthetic polypeptide"
DIQMTQSPSTLSASVGDRVTITCRASQSIRSWLAWYQQKPGKAPKLLIYKASSLESGVPSRFSGSGSGTEFTLTISSLQPDDFATYYCQQYNSYSYTFGQGTKLEIKRTVAAPSVFIFPPSDEQLKSGTASVVCLLNNFYPREAKVQWKVDNALQSGNSQESVTEQDSKDSTYSLSSTLTLSKADYEKHKVYACEVTHQGLSSPVTKSFNRGEC

SEQ ID NO: 27 - protein, 247 aa, synthetic construct
  SITE 227..247: note = /note="This region may be absent in its entirety"
  VARIANT 230: note = L
  SITE 231..247: note = /note="This region may be absent in its entirety"
  SITE 237..247: note = /note="This region may be absent in its entirety"
  SITE 1..247: note = /note="Variant residues given in the sequence have no preference with respect to those in the annotations for variant positions"
  REGION 1..247: note = source = /note="Description of Artificial Sequence: Synthetic polypeptide"
  REGION 1..247: note = source = /note="See specification as filed for detailed description of substitutions and preferred embodiments"
EVQLLESGGGLVQPGGSLRLSCAASGFTFSSYAMSWVRQAPGKGLEWVSGITGSGGSTYYADSVKGRFTISRDNSKNTLYLQMNSLRAEDTAVYYCAKDPGTTVIMSWFDPWGQGTLVTVSSASTKGPSVFPLAPSSKSTSGGTAALGCLVKDYFPEPVTVSWNSGALTSGVHTFPAVLQSSGLYSLSSVVTVPSSSLGTQTYICNVNHKPSNTKVDKKVEPKSCDKTHTCPPCPAPELLGGPSVFL

SEQ ID NO: 28 - protein, 215 aa, synthetic construct
  REGION 1..215: note = source = /note="Description of Artificial Sequence: Synthetic polypeptide"
EIVLTQSPGTLSLSPGERATLSCRASQSVRGRYLAWYQQKPGQAPRLLIYGASSRATGIPDRFSGSGSGTDFTLTISRLEPEDFAVFYCQQYGSSPRTFGQGTKVEIKRTVAAPSVFIFPPSDEQLKSGTASVVCLLNNFYPREAKVQWKVDNALQSGNSQESVTEQDSKDSTYSLSSTLTLSKADYEKHKVYACEVTHQGLSSPVTKSFNRGEC

SEQ ID NO: 29 - protein, 235 aa, synthetic construct
  SITE 216..235: note = /note="This region may be absent in its entirety"
  SITE 225..235: note = /note="This region may be absent in its entirety"
  SITE 1..235: note = /note="Variant residues given in the sequence have no preference with respect to those in the annotations for variant positions"
  REGION 1..235: note = source = /note="Description of Artificial Sequence: Synthetic polypeptide"
  REGION 1..235: note = source = /note="See specification as filed for detailed description of substitutions and preferred embodiments"
QVQLVESGGGVVQPGRSLRLDCKASGITFSNSGMHWVRQAPGKGLEWVAVIWYDGSKRYYADSVKGRFTISRDNSKNTLFLQMNSLRAEDTAVYYCATNDDYWGQGTLVTVSSASTKGPSVFPLAPCSRSTSESTAALGCLVKDYFPEPVTVSWNSGALTSGVHTFPAVLQSSGLYSLSSVVTVPSSSLGTKTYTCNVDHKPSNTKVDKRVESKYGPPCPPCPAPEFLGGPSVFL

SEQ ID NO: 30 - protein, 214 aa, synthetic construct
  REGION 1..214: note = source = /note="Description of Artificial Sequence: Synthetic polypeptide"
EIVLTQSPATLSLSPGERATLSCRASQSVSSYLAWYQQKPGQAPRLLIYDASNRATGIPARFSGSGSGTDFTLTISSLEPEDFAVYYCQQSSNWPRTFGQGTKVEIKRTVAAPSVFIFPPSDEQLKSGTASVVCLLNNFYPREAKVQWKVDNALQSGNSQESVTEQDSKDSTYSLSSTLTLSKADYEKHKVYACEVTHQGLSSPVTKSFNRGEC

SEQ ID NO: 31 - protein, 242 aa, synthetic construct
  SITE 223..242: note = /note="This region may be absent in its entirety"
  SITE 232..242: note = /note="This region may be absent in its entirety"
  SITE 1..242: note = /note="Variant residues given in the sequence have no preference with respect to those in the annotations for variant positions"
  REGION 1..242: note = source = /note="Description of Artificial Sequence: Synthetic polypeptide"
  REGION 1..242: note = source = /note="See specification as filed for detailed description of substitutions and preferred embodiments"
QVQLVQSGVEVKKPGASVKVSCKASGYTFTNYYMYWVRQAPGQGLEWMGGINPSNGGTNFNEKFKNRVTLTTDSSTTTAYMELKSLQFDDTAVYYCARRDYRFDMGFDYWGQGTTVTVSSASTKGPSVFPLAPCSRSTSESTAALGCLVKDYFPEPVTVSWNSGALTSGVHTFPAVLQSSGLYSLSSVVTVPSSSLGTKTYTCNVDHKPSNTKVDKRVESKYGPPCPPCPAPEFLGGPSVFL

SEQ ID NO: 32 - protein, 218 aa, synthetic construct
  REGION 1..218: note = source = /note="Description of Artificial Sequence: Synthetic polypeptide"
EIVLTQSPATLSLSPGERATLSCRASKGVSTSGYSYLHWYQQKPGQAPRLLIYLASYLESGVPARFSGSGSGTDFTLTISSLEPEDFAVYYCQHSRDLPLTFGGGTKVEIKRTVAAPSVFIFPPSDEQLKSGTASVVCLLNNFYPREAKVQWKVDNALQSGNSQESVTEQDSKDSTYSLSSTLTLSKADYEKHKVYACEVTHQGLSSPVTKSFNRGEC

SEQ ID NO: 33 - protein, 248 aa, synthetic construct
  SITE 228..248: note = /note="This region may be absent in its entirety"
  VARIANT 231: note = L
  SITE 232..248: note = /note="This region may be absent in its entirety"
  SITE 238..248: note = /note="This region may be absent in its entirety"
  SITE 1..248: note = /note="Variant residues given in the sequence have no preference with respect to those in the annotations for variant positions"
  REGION 1..248: note = source = /note="Description of Artificial Sequence: Synthetic polypeptide"
  REGION 1..248: note = source = /note="See specification as filed for detailed description of substitutions and preferred embodiments"
EVQLVESGGGLVQPGGSLRLSCAASGYDFTHYGMNWVRQAPGKGLEWVGWINTYTGEPTYAADFKRRFTFSLDTSKSTAYLQMNSLRAEDTAVYYCAKYPYYYGTSHWYFDVWGQGTLVTVSSASTKGPSVFPLAPSSKSTSGGTAALGCLVKDYFPEPVTVSWNSGALTSGVHTFPAVLQSSGLYSLSSVVTVPSSSLGTQTYICNVNHKPSNTKVDKKVEPKSCDKTHTCPPCPAPELLGGPSVFL

SEQ ID NO: 34 - protein, 214 aa, synthetic construct
  REGION 1..214: note = source = /note="Description of Artificial Sequence: Synthetic polypeptide"
DIQLTQSPSSLSASVGDRVTITCSASQDISNYLNWYQQKPGKAPKVLIYFTSSLHSGVPSRFSGSGSGTDFTLTISSLQPEDFATYYCQQYSTVPWTFGQGTKVEIKRTVAAPSVFIFPPSDEQLKSGTASVVCLLNNFYPREAKVQWKVDNALQSGNSQESVTEQDSKDSTYSLSSTLTLSKADYEKHKVYACEVTHQGLSSPVTKSFNRGEC

SEQ ID NO: 35 - protein, 248 aa, synthetic construct
  SITE 228..248: note = /note="This region may be absent in its entirety"
  VARIANT 231: note = L
  SITE 232..248: note = /note="This region may be absent in its entirety"
  SITE 238..248: note = /note="This region may be absent in its entirety"
  SITE 1..248: note = /note="Variant residues given in the sequence have no preference with respect to those in the annotations for variant positions"
  REGION 1..248: note = source = /note="Description of Artificial Sequence: Synthetic polypeptide"
  REGION 1..248: note = source = /note="See specification as filed for detailed description of substitutions and preferred embodiments"
EVQLVESGGGLVQPGGSLRLSCAASGYTFTNYGMNWVRQAPGKGLEWVGWINTYTGEPTYAADFKRRFTFSLDTSKSTAYLQMNSLRAEDTAVYYCAKYPHYYGSSHWYFDVWGQGTLVTVSSASTKGPSVFPLAPSSKSTSGGTAALGCLVKDYFPEPVTVSWNSGALTSGVHTFPAVLQSSGLYSLSSVVTVPSSSLGTQTYICNVNHKPSNTKVDKKVEPKSCDKTHTCPPCPAPELLGGPSVFL

SEQ ID NO: 36 - protein, 214 aa, synthetic construct
  REGION 1..214: note = source = /note="Description of Artificial Sequence: Synthetic polypeptide"
DIQMTQSPSSLSASVGDRVTITCSASQDISNYLNWYQQKPGKAPKVLIYFTSSLHSGVPSRFSGSGSGTDFTLTISSLQPEDFATYYCQQYSTVPWTFGQGTKVEIKRTVAAPSVFIFPPSDEQLKSGTASVVCLLNNFYPREAKVQWKVDNALQSGNSQESVTEQDSKDSTYSLSSTLTLSKADYEKHKVYACEVTHQGLSSPVTKSFNRGEC

SEQ ID NO: 37 - protein, 240 aa, synthetic construct
  SITE 220..240: note = /note="This region may be absent in its entirety"
  VARIANT 223: note = L
  SITE 224..240: note = /note="This region may be absent in its entirety"
  SITE 230..240: note = /note="This region may be absent in its entirety"
  SITE 1..240: note = /note="Variant residues given in the sequence have no preference with respect to those in the annotations for variant positions"
  REGION 1..240: note = source = /note="Description of Artificial Sequence: Synthetic polypeptide"
  REGION 1..240: note = source = /note="See specification as filed for detailed description of substitutions and preferred embodiments"
EVQLVQSGPELKKPGASVKVSCKASGYTFTNYGMNWVRQAPGQGLEWMGWINTYTGETTYADDFKGRFVFSLDTSVSTAYLQISSLKAEDTAVYYCEREGGVNNWGQGTLVTVSSASTKGPSVFPLAPSSKSTSGGTAALGCLVKDYFPEPVTVSWNSGALTSGVHTFPAVLQSSGLYSLSSVVTVPSSSLGTQTYICNVNHKPSNTKVDKKVEPKSCDKTHTCPPCPAPELLGGPSVFL

SEQ ID NO: 38 - protein, 214 aa, synthetic construct
  REGION 1..214: note = source = /note="Description of Artificial Sequence: Synthetic polypeptide"
DIQVTQSPSSLSASVGDRVTITCITSTDIDDDMNWYQQKPGKVPKLLISGGNTLRPGVPSRFSGSGSGTDFTLTISSLQPEDVATYYCLQSDSLPYTFGQGTKVEIKRTVAAPSVFIFPPSDEQLKSGTASVVCLLNNFYPREAKVQWKVDNALQSGNSQESVTEQDSKDSTYSLSSTLTLSKADYEKHKVYACEVTHQGLSSPVTKSFNRGEC

SEQ ID NO: 39 - protein, 120 aa, synthetic construct
  REGION 1..120: note = source = /note="Description of Artificial Sequence: Synthetic polypeptide"
EVQLVESGGGLVQPGGSLRLSCTASGFSLTDYYYMTWVRQAPGKGLEWVGFIDPDDDPYYATWAKGRFTISRDNSKNTLYLQMNSLRAEDTAVYYCAGGDHNSGWGLDIWGQGTLVTVSS

SEQ ID NO: 40 - protein, 111 aa, synthetic construct
  REGION 1..111: note = source = /note="Description of Artificial Sequence: Synthetic polypeptide"
EIVMTQSPSTLSASVGDRVIITCQASEIIHSWLAWYQQKPGKAPKLLIYLASTLASGVPSRFSGSGSGAEFTLTISSLQPDDFATYYCQNVYLASTNGANFGQGTKLTVLG

SEQ ID NO: 41 - protein, 248 aa, synthetic construct
  SITE 228..248: note = /note="This region may be absent in its entirety"
  VARIANT 231: note = L
  SITE 232..248: note = /note="This region may be absent in its entirety"
  SITE 238..248: note = /note="This region may be absent in its entirety"
  SITE 1..248: note = /note="Variant residues given in the sequence have no preference with respect to those in the annotations for variant positions"
  REGION 1..248: note = source = /note="Description of Artificial Sequence: Synthetic polypeptide"
  REGION 1..248: note = source = /note="See specification as filed for detailed description of substitutions and preferred embodiments"
QVQLQQSGAEVKKPGSSVRVSCKASGGTFNNNAINWVRQAPGQGLEWMGGIIPMFGTAKYSQNFQGRVAITADESTGTASMELSSLRSEDTAVYYCARSRDLLLFPHHALSPWGRGTMVTVSSASTKGPSVFPLAPSSKSTSGGTAALGCLVKDYFPEPVTVSWNSGALTSGVHTFPAVLQSSGLYSLSSVVTVPSSSLGTQTYICNVNHKPSNTKVDKKVEPKSCDKTHTCPPCPAPELLGGPSVFL

SEQ ID NO: 42 - protein, 214 aa, synthetic construct
  REGION 1..214: note = source = /note="Description of Artificial Sequence: Synthetic polypeptide"
SSELTQDPAVSVALGQTVRVTCQGDSLRSYYASWYQQKPGQAPVLVIYGKNNRPSGIPDRFSGSSSGNTASLTITGAQAEDEADYYCSSRDSSGNHWVFGGGTELTVLGQPKAAPSVTLFPPSSEELQANKATLVCLISDFYPGAVTVAWKADSSPVKAGVETTTPSKQSNNKYAASSYLSLTPEQWKSHRSYSCQVTHEGSTVEKTVAPTECS

SEQ ID NO: 43 - protein, 238 aa, synthetic construct
  SITE 228..238: note = /note="This region may be absent in its entirety"
  SITE 234..238: note = /note="This region may be absent in its entirety"
  SITE 1..238: note = /note="Variant residues given in the sequence have no preference with respect to those in the annotations for variant positions"
  REGION 1..238: note = source = /note="Description of Artificial Sequence: Synthetic polypeptide"
  REGION 1..238: note = source = /note="See specification as filed for detailed description of substitutions and preferred embodiments"
QVQLVQSGAEVKKPGASVKVSCKASGYIFSNYWIQWVRQAPGQGLEWMGEILPGSGSTEYTENFKDRVTMTRDTSTSTVYMELSSLRSEDTAVYYCARYFFGSSPNWYFDVWGQGTLVTVSSASTKGPSVFPLAPCSRSTSESTAALGCLVKDYFPEPVTVSWNSGALTSGVHTFPAVLQSSGLYSLSSVVTVPSSNFGTQTYTCNVDHKPSNTKVDKTVERKCCVECPPCPAPPVAG

SEQ ID NO: 44 - protein, 214 aa, synthetic construct [sequence omitted]

SEQ ID NO: 45 - protein, 237 aa, synthetic construct
  SITE 218..237: note = /note="This region may be absent in its entirety"
  SITE 227..237: note = /note="This region may be absent in its entirety"
  SITE 1..237: note = /note="Variant residues given in the sequence have no preference with respect to those in the annotations for variant positions"
  REGION 1..237: note = source = /note="Description of Artificial Sequence: Synthetic polypeptide"
  REGION 1..237: note = source = /note="See specification as filed for detailed description of substitutions and preferred embodiments"
QVQLQESGPGLVKPSETLSLTCTVSGFSLLSYGVHWVRQPPGKGLEWLGVIWTGGTTNYNSALMSRFTISKDDSKNTVYLKMNSLKTEDTAIYYCARYYYGMDYWGQGTLVTVSSASTKGPSVFPLAPCSRSTSESTAALGCLVKDYFPEPVTVSWNSGALTSGVHTFPAVLQSSGLYSLSSVVTVPSSSLGTKTYTCNVDHKPSNTKVDKRVESKYGPPCPPCPAPEFLGGPSVFL

SEQ ID NO: 46 - protein, 214 aa, synthetic construct
  REGION 1..214: note = source = /note="Description of Artificial Sequence: Synthetic polypeptide"
DIQMTQSPSSLSASVGDRVTITCKASQDVRNTVAWYQQKPGKAPKLLIYSSSYRNTGVPDRFSGSGSGTDFTLTISSLQAEDVAVYYCQQHYITPYTFGGGTKVEIKRTVAAPSVFIFPPSDEQLKSGTASVVCLLNNFYPREAKVQWKVDNALQSGNSQESVTEQDSKDSTYSLSSTLTLSKADYEKHKVYACEVTHQGLSSPVTKSFNRGEC

SEQ ID NO: 47 - protein, 247 aa, synthetic construct
  SITE 227..247: note = /note="This region may be absent in its entirety"
  VARIANT 230: note = L
  SITE 231..247: note = /note="This region may be absent in its entirety"
  SITE 237..247: note = /note="This region may be absent in its entirety"
  SITE 1..247: note = /note="Variant residues given in the sequence have no preference with respect to those in the annotations for variant positions"
  REGION 1..247: note = source = /note="Description of Artificial Sequence: Synthetic polypeptide"
  REGION 1..247: note = source = /note="See specification as filed for detailed description of substitutions and preferred embodiments"
EVQLLESGGGLVQPGGSLRLSCAASGFTFSHYIMMWVRQAPGKGLEWVSGIYSSGGITVYADSVKGRFTISRDNSKNTLYLQMNSLRAEDTAVYYCAYRRIGVPRRDEFDIWGQGTMVTVSSASTKGPSVFPLAPSSKSTSGGTAALGCLVKDYFPEPVTVSWNSGALTSGVHTFPAVLQSSGLYSLSSVVTVPSSSLGTQTYICNVNHKPSNTKVDKRVEPKSCDKTHTCPPCPAPELLGGPSVFL

SEQ ID NO: 48 - protein, 213 aa, synthetic construct
  REGION 1..213: note = source = /note="Description of Artificial Sequence: Synthetic polypeptide"
DIQMTQSPSTLSASVGDRVTITCRASQSISSWLAWYQQKPGKAPKLLIYKASTLESGVPSRFSGSGSGTEFTLTISSLQPDDFATYYCQQYNTYWTFGQGTKVEIKRTVAAPSVFIFPPSDEQLKSGTASVVCLLNNFYPREAKVQWKVDNALQSGNSQESVTEQDSKDSTYSLSSTLTLSKADYEKHKVYACEVTHQGLSSPVTKSFNRGEC

SEQ ID NO: 49 - protein, 246 aa, synthetic construct
  SITE 226..246: note = /note="This region may be absent in its entirety"
  VARIANT 229: note = L
  SITE 230..246: note = /note="This region may be absent in its entirety"
  SITE 236..246: note = /note="This region may be absent in its entirety"
  SITE 1..246: note = /note="Variant residues given in the sequence have no preference with respect to those in the annotations for variant positions"
  REGION 1..246: note = source = /note="Description of Artificial Sequence: Synthetic polypeptide"
  REGION 1..246: note = source = /note="See specification as filed for detailed description of substitutions and preferred embodiments"
EVQLVESGGGLVQPGRSLRLSCAASGFTFDDYAMHWVRQAPGKGLEWVSAITWNSGHIDYADSVEGRFTISRDNAKNSLYLQMNSLRAEDTAVYYCAKVSYLSTASSLDYWGQGTLVTVSSASTKGPSVFPLAPSSKSTSGGTAALGCLVKDYFPEPVTVSWNSGALTSGVHTFPAVLQSSGLYSLSSVVTVPSSSLGTQTYICNVNHKPSNTKVDKKVEPKSCDKTHTCPPCPAPELLGGPSVFL

SEQ ID NO: 50 - protein, 154 aa, synthetic construct
  REGION 1..154: note = source = /note="Description of Artificial Sequence: Synthetic polypeptide"
RFSGSGSGTDFTLTISSLQPEDVATYYCQRYNRAPYTFGQGTKVEIKRTVAAPSVFIFPPSDEQLKSGTASVVCLLNNFYPREAKVQWKVDNALQSGNSQESVTEQDSKDSTYSLSSTLTLSKADYEKHKVYACEVTHQGLSSPVTKSFNRGEC

SEQ ID NO: 51 - protein, 245 aa, synthetic construct
  SITE 225..245: note = /note="This region may be absent in its entirety"
  VARIANT 228: note = L
  SITE 229..245: note = /note="This region may be absent in its entirety"
  SITE 235..245: note = /note="This region may be absent in its entirety"
  SITE 1..245: note = /note="Variant residues given in the sequence have no preference with respect to those in the annotations for variant positions"
  REGION 1..245: note = source = /note="Description of Artificial Sequence: Synthetic polypeptide"
  REGION 1..245: note = source = /note="See specification as filed for detailed description of substitutions and preferred embodiments"
EVKLEESGGGLVQPGGSMKLSCVASGFIFSNHWMNWVRQSPEKGLEWVAEIRSKSINSATHYAESVKGRFTISRDDSKSAVYLQMTDLRTEDTGVYYCSRNYYGSTYDYWGQGTTLTVSSASTKGPSVFPLAPSSKSTSGGTAALGCLVKDYFPEPVTVSWNSGALTSGVHTFPAVLQSSGLYSLSSVVTVPSSSLGTQTYICNVNHKPSNTKVDKKVEPKSCDKTHTCPPCPAPELLGGPSVFL

SEQ ID NO: 52 - protein, 214 aa, synthetic construct
  REGION 1..214: note = source = /note="Description of Artificial Sequence: Synthetic polypeptide"
DILLTQSPAILSVSPGERVSFSCRASQFVGSSIHWYQQRTNGSPRLLIKYASESMSGIPSRFSGSGSGTDFTLSINTVESEDIADYYCQQSHSWPFTFGSGTNLEVKRTVAAPSVFIFPPSDEQLKSGTASVVCLLNNFYPREAKVQWKVDNALQSGNSQESVTEQDSKDSTYSLSSTLTLSKADYEKHKVYACEVTHQGLSSPVTKSFNRGEC

SEQ ID NO: 53 - protein, 237 aa, synthetic construct
  SITE 218..237: note = /note="This region may be absent in its entirety"
  SITE 227..237: note = /note="This region may be absent in its entirety"
  SITE 1..237: note = /note="Variant residues given in the sequence have no preference with respect to those in the annotations for variant positions"
  REGION 1..237: note = source = /note="Description of Artificial Sequence: Synthetic polypeptide"
  REGION 1..237: note = source = /note="See specification as filed for detailed description of substitutions and preferred embodiments"
EVKVVESGGGLVQPGGSMKLSCVVSGFTFSNYWVNWVRQAPGKGLEWVAQIRLKSDNYATHYEESVKGRFTISRDDSKSSVYLQMNNLRAEDSGIYYCTNWEDYWGQGTTVTVSSASTKGPSVFPLAPCSRSTSESTAALGCLVKDYFPEPVTVSWNSGALTSGVHTFPAVLQSSGLYSLSSVVTVPSSSLGTKTYTCNVDHKPSNTKVDKRVESKYGPPCPPCPAPEFLGGPSVFL

SEQ ID NO: 54 - protein, 218 aa, synthetic construct
  REGION 1..218: note = source = /note="Description of Artificial Sequence: Synthetic polypeptide"
DIVLTQSPDSLAVSLGERATISCRASQSVSTSRYSYIHWYQQKPGQPPKLLIKYASNLESGVPSRFSGSGSGTDFTLNIHPLEPEDFATYYCHHSWEIPLTFGQGTKLEIKRTVAAPSVFIFPPSDEQLKSGTASVVCLLNNFYPREAKVQWKVDNALQSGNSQESVTEQDSKDSTYSLSSTLTLSKADYEKHKVYACEVTHQGLSSPVTKSFNRGEC

SEQ ID NO: 55 - protein, 246 aa, synthetic construct
  SITE 236..246: note = /note="This region may be absent in its entirety"
  SITE 242..246: note = /note="This region may be absent in its entirety"
  SITE 1..246: note = /note="Variant residues given in the sequence have no preference with respect to those in the annotations for variant positions"
  REGION 1..246: note = source = /note="Description of Artificial Sequence: Synthetic polypeptide"
  REGION 1..246: note = source = /note="See specification as filed for detailed description of substitutions and preferred embodiments"
QVQLVESGGGVVQPGRSLRLSCAASGFTFSSFGMHWVRQAPGKGLEWVAVISFDGSIKYSVDSVKGRFTISRDNSKNTLFLQMNSLRAEDTAVYYCARDRLNYYDSSGYYHYKYYGMAVWGQGTTVTVSSASTKGPSVFPLAPCSRSTSESTAALGCLVKDYFPEPVTVSWNSGALTSGVHTFPAVLQSSGLYSLSSVVTVPSSNFGTQTYTCNVDHKPSNTKVDKTVERKCCVECPPCPAPPVAG

SEQ ID NO: 56 - protein, 216 aa, synthetic construct
  REGION 1..216: note = source = /note="Description of Artificial Sequence: Synthetic polypeptide"
QSVLTQPPSVSAAPGQKVTISCSGSSSNIGNNYVSWYQQLPGTAPKLLIYDNNKRPSGIPDRFSGSKSGTSTTLGITGLQTGDEADYYCGTWDSRLSAVVFGGGTKLTVLGQPKANPTVTLFPPSSEELQANKATLVCLISDFYPGAVTVAWKADGSPVKAGVETTKPSKQSNNKYAASSYLSLTPEQWKSHRSYSCQVTHEGSTVEKTVAPTECS

SEQ ID NO: 57 - protein, 244 aa, synthetic construct
  SITE 229..244: note = /note="This region may be absent in its entirety"
  VARIANT 232: note = L
  SITE 233..244: note = /note="This region may be absent in its entirety"
  SITE 239..244: note = /note="This region may be absent in its entirety"
  SITE 1..244: note = /note="Variant residues given in the sequence have no preference with respect to those in the annotations for variant positions"
  REGION 1..244: note = source = /note="Description of Artificial Sequence: Synthetic polypeptide"
  REGION 1..244: note = source = /note="See specification as filed for detailed description of substitutions and preferred embodiments"
EVQLVESGGGLVQPGGSLRLSCSASGFTFSSFGMHWVRQAPGKGLEWVAYISSGSSTIYYGDTVKGRFTISRDNAKNSLFLQMSSLRAEDTAVYYCAREGGYYYGRSYYTMDYWGQGTTVTVSSASTKGPSVFPLAPSSKSTSGGTAALGCLVKDYFPEPVTVSWNSGALTSGVHTFPAVLQSSGLYSLSSVVTVPSSSLGTQTYICNVNHKPSNTKVDKKVEPKSCDKTHTCPPCPAPELLGG

SEQ ID NO: 58 - protein, 219 aa, synthetic construct
  REGION 1..219: note = source = /note="Description of Artificial Sequence: Synthetic polypeptide"
DVVMTQSPLSLPVTPGAPASISCRSSQSIVHSNGNTYLEWYLQKPGQSPKLLIYKVSNRFSGVPDRFSGSGSGTDFTLRISRVEAEDVGIYYCFQGSHVPPTFGPGTKLEIKRTVAAPSVFIFPPSDEQLKSGTASVVCLLNNFYPREAKVQWKVDNALQSGNSQESVTEQDSKDSTYSLSSTLTLSKADYEKHKVYACEVTHQGLSSPVTKSFNRGEC

SEQ ID NO: 59 - protein, 123 aa, synthetic construct
  REGION 1..123: note = source = /note="Description of Artificial Sequence: Synthetic polypeptide"
EVKLVESGGGLVQPGGSLRLSCATSGFTFSDFYMEWVRQAPGKRLEWIAASRNKANDYTTEYADSVKGRFIVSRDTSQSILYLQMNALRAEDTAIYYCARDYYGSSYWYFDVWGAGTTVTVSS

SEQ ID NO: 60 - protein, 113 aa, synthetic construct
  REGION 1..113: note = source = /note="Description of Artificial Sequence: Synthetic polypeptide"
DIVMTQSPSSLSVSAGKKVTISCTASESLYSSKHKVHYLAWYQKKPEQSPKLLIYGASNRYIGVPDRFTGSGSGTDFTLTISSVQVEDLTHYYCAQFYSYPLTFGAGTKLEIK

SEQ ID NO: 61-70 - skipped (10 entries)

SEQ ID NO: 71 - protein, 736 aa, Adeno-associated virus 1
MAADGYLPDWLEDNLSEGIREWWDLKPGAPKPKANQQKQDDGRGLVLPGYKYLGPFNGLDKGEPVNAADAAALEHDKAYDQQLKAGDNPYLRYNHADAEFQERLQEDTSFGGNLGRAVFQAKKRVLEPLGLVEEGAKTAPGKKRPVEQSPQEPDSSSGIGKTGQQPAKKRLNFGQTGDSESVPDPQPLGEPPATPAAVGPTTMASGGGAPMADNNEGADGVGNASGNWHCDSTWLGDRVITTSTRTWALPTYNNHLYKQISSASTGASNDNHYFGYSTPWGYFDFNRFHCHFSPRDWQRLINNNWGFRPKRLNFKLFNIQVKEVTTNDGVTTIANNLTSTVQVFSDSEYQLPYVLGSAHQGCLPPFPADVFMIPQYGYLTLNNGSQAVGRSSFYCLEYFPSQMLRTGNNFTFSYTFEEVPFHSSYAHSQSLDRLMNPLIDQYLYYLNRTQNQSGSAQNKDLLFSRGSPAGMSVQPKNWLPGPCYRQQRVSKTKTDNNNSNFTWTGASKYNLNGRESIINPGTAMASHKDDEDKFFPMSGVMIFGKESAGASNTALDNVMITDEEEIKATNPVATERFGTVAVNFQSSSTDPATGDVHAMGALPGMVWQDRDVYLQGPIWAKIPHTDGHFHPSPLMGGFGLKNPPPQILIKNTPVPANPPAEFSATKFASFITQYSTGQVSVEIEWELQKENSKRWNPEVQYTSNYAKSANVDFTVDNNGLYTEPRPIGTRYLTRPL

SEQ ID NO: 72 - protein, 735 aa, Adeno-associated virus 2 [sequence omitted]

SEQ ID NO: 73 - protein, 736 aa, Adeno-associated virus 3
MAADGYLPDWLEDNLSEGIREWWALKPGVPQPKANQQHQDNRRGLVLPGYKYLGPGNGLDKGEPVNEADAAALEHDKAYDQQLKAGDNPYLKYNHADAEFQERLQEDTSFGGNLGRAVFQAKKRILEPLGLVEEAAKTAPGKKGAVDQSPQEPDSSSGVGKSGKQPARKRLNFGQTGDSESVPDPQPLGEPPAAPTSLGSNTMASGGGAPMADNNEGADGVGNSSGNWHCDSQWLGDRVITTSTRTWALPTYNNHLYKQISSQSGASNDNHYFGYSTPWGYFDFNRFHCHFSPRDWQRLINNNWGFRPKKLSFKLFNIQVRGVTQNDGTTTIANNLTSTVQVFTDSEYQLPYVLGSAHQGCLPPFPADVFMVPQYGYLTLNNGSQAVGRSSFYCLEYFPSQMLRTGNNFQFSYTFEDVPFHSSYAHSQSLDRLMNPLIDQYLYYLNRTQGTTSGTTNQSRLLFSQAGPQSMSLQARNWLPGPCYRQQRLSKTANDNNNSNFPWTAASKYHLNGRDSLVNPGPAMASHKDDEEKFFPMHGNLIFGKEGTTASNAELDNVMITDEEEIRTTNPVATEQYGTVANNLQSSNTAPTTGTVNHQGALPGMVWQDRDVYLQGPIWAKIPHTDGHFHPSPLMGGFGLKHPPPQIMIKNTPVPANPPTTFSPAKFASFITQYSTGQVSVEIEWELQKENSKRWNPEIQYTSNYNKSVNVDFTVDTNGVYSEPRPIGTRYLTRNL

SEQ ID NO: 74 - protein, 734 aa, Adeno-associated virus 4
MTDGYLPDWLEDNLSEGVREWWALQPGAPKPKANQQHQDNARGLVLPGYKYLGPGNGLDKGEPVNAADAAALEHDKAYDQQLKAGDNPYLKYNHADAEFQQRLQGDTSFGGNLGRAVFQAKKRVLEPLGLVEQAGETAPGKKRPLIESPQQPDSSTGIGKKGKQPAKKKLVFEDETGAGDGPPEGSTSGAMSDDSEMRAAAGGAAVEGGQGADGVGNASGDWHCDSTWSEGHVTTTSTRTWVLPTYNNHLYKRLGESLQSNTYNGFSTPWGYFDFNRFHCHFSPRDWQRLINNNWGMRPKAMRVKIFNIQVKEVTTSNGETTVANNLTSTVQIFADSSYELPYVMDAGQEGSLPPFPNDVFMVPQYGYCGLVTGNTSQQQTDRNAFYCLEYFPSQMLRTGNNFEITYSFEKVPFHSMYAHSQSLDRLMNPLIDQYLWGLQSTTTGTTLNAGTATTNFTKLRPTNFSNFKKNWLPGPSIKQQGFSKTANQNYKIPATGSDSLIKYETHSTLDGRWSALTPGPPMATAGPADSKFSNSQLIFAGPKQNGNTATVPGTLIFTSEEELAATNATDTDMWGNLPGGDQSNSNLPTVDRLTALGAVPGMVWQNRDIYYQGPIWAKIPHTDGHFHPSPLIGGFGLKHPPPQIFIKNTPVPANPATTFSSTPVNSFITQYSTGQVSVQIDWEIQKERSKRWNPEVQFTSNYGQQNSLLWAPDAAGKYTEPRAIGTRYLTHHL

SEQ ID NO: 75 - protein, 724 aa, Adeno-associated virus 5
MSFVDHPPDWLEEVGEGLREFLGLEAGPPKPKPNQQHQDQARGLVLPGYNYLGPGNGLDRGEPVNRADEVAREHDISYNEQLEAGDNPYLKYNHADAEFQEKLADDTSFGGNLGKAVFQAKKRVLEPFGLVEEGAKTAPTGKRIDDHFPKRKKARTEEDSKPSTSSDAEAGPSGSQQLQIPAQPASSLGADTMSAGGGGPLGDNNQGADGVGNASGDWHCDSTWMGDRVVTKSTRTWVLPSYNNHQYREIKSGSVDGSNANAYFGYSTPWGYFDFNRFHSHWSPRDWQRLINNYWGFRPRSLRVKIFNIQVKEVTVQDSTTTIANNLTSTVQVFTDDDYQLPYVVGNGTEGCLPAFPPQVFTLPQYGYATLNRDNTENPTERSSFFCLEYFPSKMLRTGNNFEFTYNFEEVPFHSSFAPSQNLFKLANPLVDQYLYRFVSTNNTGGVQFNKNLAGRYANTYKNWFPGPMGRTQGWNLGSGVNRASVSAFATTNRMELEGASYQVPPQPNGMTNNLQGSNTYALENTMIFNSQPANPGTTATYLEGNMLITSESETQPVNRVAYNVGGQMATNNQSSTTAPATGTYNLQEIVPGSVWMERDVYLQGPIWAKIPETGAHFHPSPAMGGFGLKHPPPMMLIKNTPVPGNITSFSDVPVSSFITQYSTGQVTVEMEWELKKENSKRWNPEIQYTNNYNDPQFVDFAPDSTGEYRTTRPIGTRYLTRPL

SEQ ID NO: 76 - protein, 736 aa, Adeno-associated virus 6
MAADGYLPDWLEDNLSEGIREWWDLKPGAPKPKANQQKQDDGRGLVLPGYKYLGPFNGLDKGEPVNAADAAALEHDKAYDQQLKAGDNPYLRYNHADAEFQERLQEDTSFGGNLGRAVFQAKKRVLEPFGLVEEGAKTAPGKKRPVEQSPQEPDSSSGIGKTGQQPAKKRLNFGQTGDSESVPDPQPLGEPPATPAAVGPTTMASGGGAPMADNNEGADGVGNASGNWHCDSTWLGDRVITTSTRTWALPTYNNHLYKQISSASTGASNDNHYFGYSTPWGYFDFNRFHCHFSPRDWQRLINNNWGFRPKRLNFKLFNIQVKEVTTNDGVTTIANNLTSTVQVFSDSEYQLPYVLGSAHQGCLPPFPADVFMIPQYGYLTLNNGSQAVGRSSFYCLEYFPSQMLRTGNNFTFSYTFEDVPFHSSYAHSQSLDRLMNPLIDQYLYYLNRTQNQSGSAQNKDLLFSRGSPAGMSVQPKNWLPGPCYRQQRVSKTKTDNNNSNFTWTGASKYNLNGRESIINPGTAMASHKDDKDKFFPMSGVMIFGKESAGASNTALDNVMITDEEEIKATNPVATERFGTVAVNLQSSSTDPATGDVHVMGALPGMVWQDRDVYLQGPIWAKIPHTDGHFHPSPLMGGFGLKHPPPQILIKNTPVPANPPAEFSATKFASFITQYSTGQVSVEIEWELQKENSKRWNPEVQYTSNYAKSANVDFTVDNNGLYTEPRPIGTRYLTRPL

SEQ ID NO: 77 - protein, 737 aa, Adeno-associated virus 7
MAADGYLPDWLEDNLSEGIREWWDLKPGAPKPKANQQKQDNGRGLVLPGYKYLGPFNGLDKGEPVNAADAAALEHDKAYDQQLKAGDNPYLRYNHADAEFQERLQEDTSFGGNLGRAVFQAKKRVLEPLGLVEEGAKTAPAKKRPVEPSPQRSPDSSTGIGKKGQQPARKRLNFGQTGDSESVPDPQPLGEPPAAPSSVGSGTVAAGGGAPMADNNEGADGVGNASGNWHCDSTWLGDRVITTSTRTWALPTYNNHLYKQISSETAGSTNDNTYFGYSTPWGYFDFNRFHCHFSPRDWQRLINNNWGFRPKKLRFKLFNIQVKEVTTNDGVTTIANNLTSTIQVFSDSEYQLPYVLGSAHQGCLPPFPADVFMIPQYGYLTLNNGSQSVGRSSFYCLEYFPSQMLRTGNNFEFSYSFEDVPFHSSYAHSQSLDRLMNPLIDQYLYYLARTQSNPGGTAGNRELQFYQGGPSTMAEQAKNWLPGPCFRQQRVSKTLDQNNNSNFAWTGATKYHLNGRNSLVNPGVAMATHKDDEDRFFPSSGVLIFGKTGATNKTTLENVLMTNEEEIRPTNPVATEEYGIVSSNLQAANTAAQTQVVNNQGALPGMVWQNRDVYLQGPIWAKIPHTDGNFHPSPLMGGFGLKHPPPQILIKNTPVPANPPEVFTPAKFASFITQYSTGQVSVEIEWELQKENSKRWNPEIQYTSNFEKQTGVDFAVDSQGVYSEPRPIGTRYLTRNL

SEQ ID NO: 78 - protein, 738 aa, Adeno-associated virus 8
MAADGYLPDWLEDNLSEGIREWWALKPGAPKPKANQQKQDDGRGLVLPGYKYLGPFNGLDKGEPVNAADAAALEHDKAYDQQLQAGDNPYLRYNHADAEFQERLQEDTSFGGNLGRAVFQAKKRVLEPLGLVEEGAKTAPGKKRPVEPSPQRSPDSSTGIGKKGQQPARKRLNFGQTGDSESVPDPQPLGEPPAAPSGVGPNTMAAGGGAPMADNNEGADGVGSSSGNWHCDSTWLGDRVITTSTRTWALPTYNNHLYKQISNGTSGGATNDNTYFGYSTPWGYFDFNRFHCHFSPRDWQRLINNNWGFRPKRLSFKLFNIQVKEVTQNEGTKTIANNLTSTIQVFTDSEYQLPYVLGSAHQGCLPPFPADVFMIPQYGYLTLNNGSQAVGRSSFYCLEYFPSQMLRTGNNFQFTYTFEDVPFHSSYAHSQSLDRLMNPLIDQYLYYLSRTQTTGGTANTQTLGFSQGGPNTMANQAKNWLPGPCYRQQRVSTTTGQNNNSNFAWTAGTKYHLNGRNSLANPGIAMATHKDDEERFFPSNGILIFGKQNAARDNADYSDVMLTSEEEIKTTNPVATEEYGIVADNLQQQNTAPQIGTVNSQGALPGMVWQNRDVYLQGPIWAKIPHTDGNFHPSPLMGGFGLKHPPPQILIKNTPVPADPPTTFNQSKLNSFITQYSTGQVSVEIEWELQKENSKRWNPEIQYTSNYYKSTSVDFAVNTEGVYSEPRPIGTRYLTRNL

SEQ ID NO: 79 - protein, 736 aa, Adeno-associated virus 9
MAADGYLPDWLEDNLSEGIREWWALKPGAPQPKANQQHQDNARGLVLPGYKYLGPGNGLDKGEPVNAADAAALEHDKAYDQQLKAGDNPYLKYNHADAEFQERLKEDTSFGGNLGRAVFQAKKRLLEPLGLVEEAAKTAPGKKRPVEQSPQEPDSSAGIGKSGAQPAKKRLNFGQTGDTESVPDPQPIGEPPAAPSGVGSLTMASGGGAPVADNNEGADGVGSSSGNWHCDSQWLGDRVITTSTRTWALPTYNNHLYKQISNSTSGGSSNDNAYFGYSTPWGYFDFNRFHCHFSPRDWQRLINNNWGFRPKRLNFKLFNIQVKEVTDNNGVKTIANNLTSTVQVFTDSDYQLPYVLGSAHEGCLPPFPADVFMIPQYGYLTLNDGSQAVGRSSFYCLEYFPSQMLRTGNNFQFSYEFENVPFHSSYAHSQSLDRLMNPLIDQYLYYLSKTINGSGQNQQTLKFSVAGPSNMAVQGRNYIPGPSYRQQRVSTTVTQNNNSEFAWPGASSWALNGRNSLMNPGPAMASHKEGEDRFFPLSGSLIFGKQGTGRDNVDADKVMITNEEEIKTTNPVATESYGQVATNHQSAQAQAQTGWVQNQGILPGMVWQDRDVYLQGPIWAKIPHTDGNFHPSPLMGGFGMKHPPPQILIKNTPVPADPPTAFNKDKLNSFITQYSTGQVSVEIEWELQKENSKRWNPEIQYTSNYYKSNNVEFAVNTEGVYSEPRPIGTRYLTRNL

SEQ ID NO: 80 - protein, 738 aa, Adeno-associated virus
MAADGYLPDWLEDNLSEGIREWWDLKPGAPKPKANQQKQDDGRGLVLPGYKYLGPFNGLDKGEPVNAADAAALEHDKAYDQQLKAGDNPYLRYNHADAEFQERLQEDTSFGGNLGRAVFQAKKRVLEPLGLVEEGAKTAPGKKRPVEPSPQRSPDSSTGIGKKGQQPAKKRLNFGQTGDSESVPDPQPIGEPPAGPSGLGSGTMAAGGGAPMADNNEGADGVGSSSGNWHCDSTWLGDRVITTSTRTWALPTYNNHLYKQISNGTSGGSTNDNTYFGYSTPWGYFDFNRFHCHFSPRDWQRLINNNWGFRPKRLNFKLFNIQVKEVTQNEGTKTIANNLTSTIQVFTDSEYQLPYVLGSAHQGCLPPFPADVFMIPQYGYLTLNNGSQAVGRSSFYCLEYFPSQMLRTGNNFEFSYQFEDVPFHSSYAHSQSLDRLMNPLIDQYLYYLSRTQSTGGTAGTQQLLFSQAGPNNMSAQAKNWLPGPCYRQQRVSTTLSQNNNSNFAWTGATKYHLNGRDSLVNPGVAMATHKDDEERFFPSSGVLMFGKQGAGKDNVDYSSVMLTSEEEIKTTNPVATEQYGVVADNLQQQNAAPIVGAVNSQGALPGMVWQNRDVYLQGPIWAKIPHTDGNFHPSPLMGGFGLKHPPPQILIKNTPVPADPPTTFSQAKLASFITQYSTGQVSVEIEWELQKENSKRWNPEIQYTSNYYKSTNVDFAVNTDGTYSEPRPIGTRYLTRNL

SEQ ID NO: 81 - protein, 736 aa, Adeno-associated virus
MAADGYLPDWLEDTLSEGIRQWWKLKPGPPPPKPAERHKDDSRGLVLPGYKYLGPGNGLDKGEPVNAADAAALEHDKAYDQQLKAGDNPYLKYNHADAEFQERLKEDTSFGGNLGRAVFQAKKRLLEPLGLVEEAAKTAPGKKRPVEQSPQEPDSSAGIGKSGSQPAKKKLNFGQTGDTESVPDPQPIGEPPAAPSGVGSLTMASGGGAPVADNNEGADGVGSSSGNWHCDSQWLGDRVITTSTRTWALPTYNNHLYKQISNSTSGGSSNDNAYFGYSTPWGYFDFNRFHCHFSPRDWQRLINNNWGFRPKRLNFKLFNIQVKEVTDNNGVKTIANNLTSTVQVFTDSDYQLPYVLGSAHEGCLPPFPADVFMIPQYGYLTLNDGGQAVGRSSFYCLEYFPSQMLRTGNNFQFSYEFENVPFHSSYAHSQSLDRLMNPLIDQYLYYLSKTINGSGQNQQTLKFSVAGPSNMAVQGRNYIPGPSYRQQRVSTTVTQNNNSEFAWPGASSWALNGRNSLMNPGPAMASHKEGEDRFFPLSGSLIFGKQGTGRDNVDADKVMITNEEEIKTTNPVATESYGQVATNHQSAQAQAQTGWVQNQGILPGMVWQDRDVYLQGPIWAKIPHTDGNFHPSPLMGGFGMKHPPPQILIKNTPVPADPPTAFNKDKLNSFITQYSTGQVSVEIEWELQKENSKRWNPEIQYTSNYYKSNNVEFAVSTEGVYSEPRPIGTRYLTRNL

SEQ ID NO: 82 - protein, 736 aa, Adeno-associated virus
MAADGYLPDWLEDTLSEGIRQWWKLKPGPPPPKPAERHKDDSRGLVLPGYKYLGPGNGLDKGEPVNAADAAALEHDKAYDQQLKAGDNPYLKYNHADAEFQERLKEDTSFGGNLGRAVFQAKKRLLEPLGLVEEAAKTAPGKKRPVEQSPQEPDSSAGIGKSGSQPAKKKLNFGQTGDTESVPDPQPIGEPPAAPSGVGSLTMASGGGAPVADNNEGADGVGSSSGNWHCDSQWLGDRVITTSTRTWALPTYNNHLYKQISNSTSGGSSNDNAYFGYSTPWGYFDFNRFHCHFSPRDWQRLINNNWGFRPKRLNFKLFNIQVKEVTDNNGVKTIANNLTSTVQVFTDSDYQLPYVLGSAHEGCLPPFPADVFMIPQYGYLTLNDGSQAVGRSSFYCLEYFPSQMLRTGNNFQFSYEFENVPFHSSYAHSQSLDRLMNPLIDQYLYYLSKTINGSGQNQQTLKFSVAGPSNMAVQGRNYIPGPSYRQQRVSTTVTQNNNSEFAWPGASSWALNGRNSLMNPGPAMASHKEGEDRFFPLSGSLIFGKQGTGRDNVDADKVMITNEEEIKTTNPVATESYGQVATNHQSAQAQAQTGWVQNQGILPGMVWQDRDVYLQGPIWAKIPHTDGNFHPSPLMGGFGMKHPPPQILIKNTPVPADPPTAFNKDKLNSFITQYSTGQVSVEIEWELQKENSKRWNPEIQYTSNYYKSNNVEFAVNTEGVYSEPRPIGTRYLTRNL

SEQ ID NO: 83-100 - skipped (18 entries)

SEQ ID NO: 101 - DNA, 744 bp, synthetic construct
  misc_feature 682..744: note = /note="This region may be absent in its entirety"
  variation 691..693: replace = ctg
  misc_feature 694..744: note = /note="This region may be absent in its entirety"
  misc_feature 712..744: note = /note="This region may be absent in its entirety"
  misc_feature 1..744: note = /note="Variant nucleotides given in the sequence have no preference with respect to those in the annotations for variant positions"
  misc_feature 1..744: note = source = /note="Description of Artificial Sequence: Synthetic polynucleotide"
  misc_feature 1..744: note = source = /note="See specification as filed for detailed description of substitutions and preferred embodiments"
  source 1..744: mol_type = other DNA
gtgcagctggtggagagcggcggcggcgtggtgcagcccggcagaagcctgagactgagctgcgccgccagcggcttcgccttcagcagctacggcatgcactgggtgagacaggcccccggcaagggcctggagtgggtggccgtgatctggttcgacggcaccaagaagtactacaccgacagcgtgaagggcagattcaccatcagcagagacaacagcaagaacaccctgtacctgcagatgaacaccctgagagccgaggacaccgccgtgtactactgcgccagagacagaggcatcggcgccagaagaggcccctactacatggacgtgtggggcaagggcaccaccgtgaccgtgagcagcgccagcaccaagggccccagcgtgttccccctggcccccagcagcaagagcaccagcggcggcaccgccgccctgggctgcctggtgaaggactacttccccgagcccgtgaccgtgagctggaacagcggcgccctgaccagcggcgtgcacaccttccccgccgtgctgcagagcagcggcctgtacagcctgagcagcgtggtgaccgtgcccagcagcagcctgggcacccagacctacatctgcaacgtgaaccacaagcccagcaacaccaaggtggacaagagagtggagcccaagagctgcgacaagacccacacctgccccccctgccccgcccccgagctgctgggcggccccagcgtgttcctg

SEQ ID NO: 102 - DNA, 642 bp, synthetic construct
  misc_feature 1..642: note = source = /note="Description of Artificial Sequence: Synthetic polynucleotide"
  source 1..642: mol_type = other DNA
gacatccagatgacccagagccccagcagcctgagcgccagcgtgggcgacagagtgaccatcacctgcagagccagccagagcatcagcagctacctgaactggtaccagcagaagcccggcaaggcccccaagctgctgatctacgccgccagcagcctgcagagcggcgtgcccagcagattcagcggcagcggcagcggcaccgacttcaccctgaccatcagcagcctgcagcccgaggacttcgccacctactactgccagcagagctacagcacccccctgaccttcggcggcggcaccaaggtggagatcaagagaaccgtggccgcccccagcgtgttcatcttcccccccagcgacgagcagctgaagagcggcaccgccagcgtggtgtgcctgctgaacaacttctaccccagagaggccaaggtgcagtggaaggtggacaacgccctgcagagcggcaacagccaggagagcgtgaccgagcaggacagcaaggacagcacctacagcctgagcagcaccctgaccctgagcaaggccgactacgagaagcacaaggtgtacgcctgcgaggtgacccaccagggcctgagcagccccgtgaccaagagcttcaacagaggcgagtgc

SEQ ID NO: 103 - DNA, 702 bp, synthetic construct
  misc_feature 643..702: note = /note="This region may be absent in its entirety"
  misc_feature 670..702: note = /note="This region may be absent in its entirety"
  misc_feature 1..702: note = source = /note="Description of Artificial Sequence: Synthetic polynucleotide"
  misc_feature 1..702: note = source = /note="See specification as filed for detailed description of substitutions and preferred embodiments"
  source 1..702: mol_type = other DNA
gaggtgcagctggtggagagcggcggcggcctggtgcagcccggcggcagcctgagactgagctgcgccgccagcggcttcaccttcagcagctacggcatgagctgggtgagacaggcccccggcaagggcctggagctggtggccagcatcaacagcaacggcggcagcacctactaccccgacagcgtgaagggcagattcaccatcagcagagacaacgccaagaacagcctgtacctgcagatgaacagcctgagagccgaggacaccgccgtgtactactgcgccagcggcgactactggggccagggcaccaccgtgaccgtgagcagcgccagcaccaagggccccagcgtgttccccctggccccctgcagcagaagcaccagcgagagcaccgccgccctgggctgcctggtgaaggactacttccccgagcccgtgaccgtgagctggaacagcggcgccctgaccagcggcgtgcacaccttccccgccgtgctgcagagcagcggcctgtacagcctgagcagcgtggtgaccgtgcccagcagcagcctgggcaccaagacctacacctgcaacgtggaccacaagcccagcaacaccaaggtggacaagagagtggagagcaagtacggccccccctgccccccctgccccgcccccgagttcctgggcggccccagcgtgttcctg

SEQ ID NO: 104 - DNA, 657 bp, synthetic construct
  misc_feature 1..657: note = source = /note="Description of Artificial Sequence: Synthetic polynucleotide"
  source 1..657: mol_type = other DNA
gacatcgtgatgacccagagccccctgagcctgcccgtgacccccggcgagcccgccagcatcagctgcagaagcagccagagcctggtgtacagcaacggcgacacctacctgcactggtacctgcagaagcccggccagagcccccagctgctgatctacaaggtgagcaacagattcagcggcgtgcccgacagattcagcggcagcggcagcggcaccgacttcaccctgaagatcagcagagtggaggccgaggacgtgggcgtgtactactgcagccagagcacccacgtgccctggaccttcggccagggcaccaaggtggagatcaagagaaccgtggccgcccccagcgtgttcatcttcccccccagcgacgagcagctgaagagcggcaccgccagcgtggtgtgcctgctgaacaacttctaccccagagaggccaaggtgcagtggaaggtggacaacgccctgcagagcggcaacagccaggagagcgtgaccgagcaggacagcaaggacagcacctacagcctgagcagcaccctgaccctgagcaaggccgactacgagaagcacaaggtgtacgcctgcgaggtgacccaccagggcctgagcagccccgtgaccaagagcttcaacagaggcgagtgc

SEQ ID NO: 105 - DNA, 752 bp, synthetic construct
  misc_feature 691..752: note = /note="This region may be absent in its entirety"
  misc_feature 700..702: note = Variation - /replace="ctg"
  misc_feature 703..752: note = /note="This region may be absent in its entirety"
  misc_feature 721..752: note = /note="This region may be absent in its entirety"
  misc_feature 1..752: note = /note="Variant nucleotides given in the sequence have no preference with respect to those in the annotations for variant positions"
  misc_feature 1..752: note = source = /note="Description of Artificial Sequence: Synthetic polynucleotide"
  misc_feature 1..752: note = source = /note="See specification as filed for detailed description of substitutions and preferred embodiments"
  source 1..752: mol_type = other DNA
caggtggagctggtggagagcggcggcggcctggtgcagcccggcggcagcctgagactgagctgcgccgccagcggcttcaccttcagcagctacgccatgagctgggtgagacaggcccccggcaagggcctggagtgggtgagcgccatcaacgccagcggcaccagaacctactacgccgacagcgtgaagggcagattcaccatcagcagagacaacagcaagaacaccctgtacctgcagatgaacagcctgagagccgaggacaccgccgtgtactactgcgccagaggcaagggcaacacccacaagccctacggctacgtgagatacttcgacgtgtggggccagggcaccctggtgaccgtgagcagcgccagcaccaagggccccagcgtgttccccctggcccccagcagcaagagcaccagcggcggcaccgccgccctgggctgcctggtgaaggactacttccccgagcccgtgaccgtgagctggaacagcggcgccctgaccagcggcgtgcacaccttccccgccgtgctgcagagcagcggcctgtacagcctgagcagcgtggtgaccgtgcccagcagcagcctgggcacccagacctacatctgcaacgtgaaccacaagcccagcaacaccaaggtggacaagaaggtggagcccaagagctgcgacaagacccacacctgccccccctgccccgccccgagctgctgggcggccccagcgtgttcctg

SEQ ID NO: 106 - DNA, 645 bp, synthetic construct
  misc_feature 1..645: note = source = /note="Description of Artificial Sequence: Synthetic polynucleotide"
  source 1..645: mol_type = other DNA
gacatcgtgctgacccagagccccgccaccctgagcctgagccccggcgagagagccaccctgagctgcagagccagccagagcgtgagcagcagctacctggcctggtaccagcagaagcccggccaggcccccagactgctgatctacggcgccagcagcagagccaccggcgtgcccgccagattcagcggcagcggcagcggcaccgacttcaccctgaccatcagcagcctggagcccgaggacttcgccacctactactgcctgcagatctacaacatgcccatcaccttcggccagggcaccaaggtggagatcaagagaaccgtggccgcccccagcgtgttcatcttcccccccagcgacgagcagctgaagagcggcaccgccagcgtggtgtgcctgctgaacaacttctaccccagagaggccaaggtgcagtggaaggtggacaacgccctgcagagcggcaacagccaggagagcgtgaccgagcaggacagcaaggacagcacctacagcctgagcagcaccctgaccctgagcaaggccgactacgagaagcacaaggtgtacgcctgcgaggtgacccaccagggcctgagcagccccgtgaccaagagcttcaacagaggcgagtgc

SEQ ID NO: 107 - DNA, 741 bp, synthetic construct
  misc_feature 682..741: note = /note="This region may be absent in its entirety"
  misc_feature 709..741: note = /note="This region may be absent in its entirety"
  misc_feature 1..741: note = source = /note="Description of Artificial Sequence: Synthetic polynucleotide"
  misc_feature 1..741: note = source = /note="See specification as filed for detailed description of substitutions and preferred embodiments"
  source 1..741: mol_type = other DNA
gaggtgcagctggtggagagcggcggcggcctggagcagcccggcggcagcctgagactgagctgcgccggcagcggcttcaccttcagagactacgccatgacctgggtgagacaggcccccggcaagggcctggagtgggtgagcagcatcagcggcagcggcggcaacacctactacgccgacagcgtgaagggcagattcaccatcagcagagacaacagcaagaacaccctgtacctgcagatgaacagcctgagagccgaggacaccgccgtgtactactgcgccaaggacagactgagcatcaccatcagacccagatactacggcctggacgtgtggggccagggcaccaccgtgaccgtgagcagcgccagcaccaagggccccagcgtgttccccctggccccctgcagcagaagcaccagcgagagcaccgccgccctgggctgcctggtgaaggactacttccccgagcccgtgaccgtgagctggaacagcggcgccctgaccagcggcgtgcacaccttccccgccgtgctgcagagcagcggcctgtacagcctgagcagcgtggtgaccgtgcccagcagcagcctgggcaccaagacctacacctgcaacgtggaccacaagcccagcaacaccaaggtggacaagagagtggagagcaagtacggccccccctgccccccctgccccgcccccgagttcctgggcggccccagcgtgttcctg

SEQ ID NO: 108 - DNA, 657 bp, synthetic construct
  misc_feature 1..657: note = source = /note="Description of Artificial Sequence: Synthetic polynucleotide"
  source 1..657: mol_type = other DNA
gacatcgtgatgacccagagccccctgagcctgcccgtgacccccggcgagcccgccagcatcagctgcagaagcagccagagcctgctgtacagcatcggctacaactacctggactggtacctgcagaagagcggccagagcccccagctgctgatctacctgggcagcaacagagccagcggcgtgcccgacagattcagcggcagcggcagcggcaccgacttcaccctgaagatcagcagagtggaggccgaggacgtgggcttctactactgcatgcaggccctgcagaccccctacaccttcggccagggcaccaagctggagatcaagagaaccgtggccgcccccagcgtgttcatcttcccccccagcgacgagcagctgaagagcggcaccgccagcgtggtgtgcctgctgaacaacttctaccccagagaggccaaggtgcagtggaaggtggacaacgccctgcagagcggcaacagccaggagagcgtgaccgagcaggacagcaaggacagcacctacagcctgagcagcaccctgaccctgagcaaggccgactacgagaagcacaaggtgtacgcctgcgaggtgacccaccagggcctgagcagccccgtgaccaagagcttcaacagaggcgagtgc

SEQ ID NO: 109 - DNA, 723 bp, synthetic construct
  misc_feature 664..723: note = /note="This region may be absent in its entirety"
  misc_feature 691..723: note = /note="This region may be absent in its entirety"
  misc_feature 1..723: note = source = /note="Description of Artificial Sequence: Synthetic polynucleotide"
  misc_feature 1..723: note = source = /note="See specification as filed for detailed description of substitutions and preferred embodiments"
  source 1..723: mol_type = other DNA
caggtgcagctggtgcagagcggcgccgaggtgaagaagcccggcagcagcgtgaaggtgagctgcaaggccagcggctacagcttcaccgactaccacatccactgggtgagacaggcccccggccagggcctggagtggatgggcgtgatcaaccccatgtacggcaccaccgactacaaccagagattcaagggcagagtgaccatcaccgccgacgagagcaccagcaccgcctacatggagctgagcagcctgagaagcgaggacaccgccgtgtactactgcgccagatacgactacttcaccggcaccggcgtgtactggggccagggcaccctggtgaccgtgagcagcgccagcaccaagggccccagcgtgttccccctggccccctgcagcagaagcaccagcgagagcaccgccgccctgggctgcctggtgaaggactacttccccgagcccgtgaccgtgagctggaacagcggcgccctgaccagcggcgtgcacaccttccccgccgtgctgcagagcagcggcctgtacagcctgagcagcgtggtgaccgtgcccagcagcagcctgggcaccaagacctacacctgcaacgtggaccacaagcccagcaacaccaaggtggacaagagagtggagagcaagtacggccccccctgccccccctgccccgcccccgagttcctgggcggccccagcgtgttcctg

SEQ ID NO: 110 - DNA, 657 bp, synthetic construct
  misc_feature 1..657: note = source = /note="Description of Artificial Sequence: Synthetic polynucleotide"
  source 1..657: mol_type = other DNA
gacatcgtgatgacccagacccccctgagcctgagcgtgacccccggccagcccgccagcatcagctgcagaagcagcagaagcctggtgcacagcagaggcaacacctacctgcactggtacctgcagaagcccggccagagcccccagctgctgatctacaaggtgagcaacagattcatcggcgtgcccgacagattcagcggcagcggcagcggcaccgacttcaccctgaagatcagcagagtggaggccgaggacgtgggcgtgtactactgcagccagagcacccacctgcccttcaccttcggccagggcaccaagctggagatcaagagaaccgtggccgcccccagcgtgttcatcttcccccccagcgacgagcagctgaagagcggcaccgccagcgtggtgtgcctgctgaacaacttctaccccagagaggccaaggtgcagtggaaggtggacaacgccctgcagagcggcaacagccaggagagcgtgaccgagcaggacagcaaggacagcacctacagcctgagcagcaccctgaccctgagcaaggccgactacgagaagcacaaggtgtacgcctgcgaggtgacccaccagggcctgagcagccccgtgaccaagagcttcaacagaggcgagtgc

SEQ ID NO: 111 - DNA, 755 bp, synthetic construct
  misc_feature 694..755: note = /note="This region may be absent in its entirety"
  variation 703..705: replace = ctg
  misc_feature 706..755: note = /note="This region may be absent in its entirety"
  misc_feature 724..755: note = /note="This region may be absent in its entirety"
  misc_feature 1..755: note = /note="Variant nucleotides given in the sequence have no preference with respect to those in the annotations for variant positions"
  misc_feature 1..755: note = source = /note="Description of Artificial Sequence: Synthetic polynucleotide"
  misc_feature 1..755: note = source = /note="See specification as filed for detailed description of substitutions and preferred embodiments"
  source 1..755: mol_type = other DNA
gaggtgcagctggtggagagcggcggcggcctggtgcagcccggcggcagcctgagactgagctgcgccgccagcggcttcaccttcagcaactactggatgaactgggtgagacaggcccccggcaagggcctggagtgggtggccgccatcaaccaggacggcagcgagaagtactacgtgggcagcgtgaagggcagattcaccatcagcagagacaacgccaagaacagcctgtacctgcagatgaacagcctgagagtggaggacaccgccgtgtactactgcgtgagagactactacgacatcctgaccgactactacatccactactggtacttcgacctgtggggcagaggcaccctggtgaccgtgagcagcgccagcaccaagggccccagcgtgttccccctggcccccagcagcaagagcaccagcggcggcaccgccgccctgggctgcctggtgaaggactacttccccgagcccgtgaccgtgagctggaacagcggcgccctgaccagcggcgtgcacaccttccccgccgtgctgcagagcagcggcctgtacagcctgagcagcgtggtgaccgtgcccagcagcagcctgggcacccagacctacatctgcaacgtgaaccacaagcccagcaacaccaaggtggacaagagagtggagcccaagagctgcgacaagacccacacctgccccccctgccccgccccgagctgctgggcggccccagcgtgttcctg

SEQ ID NO: 112 - DNA, 645 bp, synthetic construct
  misc_feature 1..645: note = source = /note="Description of Artificial Sequence: Synthetic polynucleotide"
  source 1..645: mol_type = other DNA
gagatcgtgctgacccagagccccggcaccctgagcctgagccccggcgagagagccaccctgagctgcagagccagccagagcgtgagcagcagctacctggcctggtaccagcagaagcccggccaggcccccagactgctgatctacggcgccagcagcagagccaccggcatccccgacagattcagcggcagcggcagcggcaccgacttcaccctgaccatcagcagactggagcccgaggacttcgccgtgtactactgccagcagtacggcagcagcccctgcaccttcggccagggcaccagactggagatcaagagaaccgtggccgcccccagcgtgttcatcttcccccccagcgacgagcagctgaagagcggcaccgccagcgtggtgtgcctgctgaacaacttctaccccagagaggccaaggtgcagtggaaggtggacaacgccctgcagagcggcaacagccaggagagcgtgaccgagcaggacagcaaggacagcacctacagcctgagcagcaccctgaccctgagcaaggccgactacgagaagcacaaggtgtacgcctgcgaggtgacccaccagggcctgagcagccccgtgaccaagagcttcaacagaggcgagtgc

SEQ ID NO: 113 - DNA, 732 bp, synthetic construct
  misc_feature 670..732: note = /note="This region may be absent in its entirety"
  variation 679..681: replace = ctg
  misc_feature 682..732: note = /note="This region may be absent in its entirety"
  misc_feature 700..732: note = /note="This region may be absent in its entirety"
  misc_feature 1..732: note = /note="Variant nucleotides given in the sequence have no preference with respect to those in the annotations for variant positions"
  misc_feature 1..732: note = source = /note="Description of Artificial Sequence: Synthetic polynucleotide"
  misc_feature 1..732: note = source = /note="See specification as filed for detailed description of substitutions and preferred embodiments"
  source 1..732: mol_type = other DNA
gaggtgcagctggtgcagagcggcgccgaggtgaagaagcccggcgagagcctgaagatcagctgcaagggcagcggctacagcttcaccacctactggctgggctgggtgagacagatgcccggcaagggcctggactggatcggcatcatgagccccgtggacagcgacatcagatacagccccagcttccagggccaggtgaccatgagcgtggacaagagcatcaccaccgcctacctgcagtggaacagcctgaaggccagcgacaccgccatgtactactgcgccagaagaagacccggccagggctacttcgacttctggggccagggcaccctggtgaccgtgagcagcagcagcaccaagggccccagcgtgttccccctggcccccagcagcaagagcaccagcggcggcaccgccgccctgggctgcctggtgaaggactacttccccgagcccgtgaccgtgagctggaacagcggcgccctgaccagcggcgtgcacaccttccccgccgtgctgcagagcagcggcctgtacagcctgagcagcgtggtgaccgtgcccagcagcagcctgggcacccagacctacatctgcaacgtgaaccacaagcccagcaacaccaaggtggacaagagagtggagcccaagagctgcgacaagacccacacctgccccccctgccccgcccccgagctgctgggcggccccagcgtgttcctg

SEQ ID NO: 114 - DNA, 642 bp, synthetic construct
  misc_feature 1..642: note = source = /note="Description of Artificial Sequence: Synthetic polynucleotide"
  source 1..642: mol_type = other DNA
gacatccagatgacccagagccccagcagcctgagcgccagcgtgggcgacagagtgaccatcacctgcagagccagccagggcatcagcagctggctggcctggtaccagcagaagcccgagaaggcccccaagagcctgatctacgccgccagcagcctgcagagcggcgtgcccagcagattcagcggcagcggcagcggcaccgacttcaccctgaccatcagcagcctgcagcccgaggacttcgccacctactactgccagcagtacaacatctacccctacaccttcggccagggcaccaagctggagatcaagagaaccgtggccgcccccagcgtgttcatcttcccccccagcgacgagcagctgaagagcggcaccgccagcgtggtgtgcctgctgaacaacttctaccccagagaggccaaggtgcagtggaaggtggacaacgccctgcagagcggcaacagccaggagagcgtgaccgagcaggacagcaaggacagcacctacagcctgagcagcaccctgaccctgagcaaggccgactacgagaagcacaaggtgtacgcctgcgaggtgacccaccagggcctgagcagccccgtgaccaagagcttcaacagaggcgagtgc

SEQ ID NO: 115 - DNA, 732 bp, synthetic construct
  misc_feature 670..732: note = /note="This region may be absent in its entirety"
  variation 679..681: replace = ctg
  misc_feature 682..732: note = /note="This region may be absent in its entirety"
  misc_feature 700..732: note = /note="This region may be absent in its entirety"
  misc_feature 1..732: note = /note="Variant nucleotides given in the sequence have no preference with respect to those in the annotations for variant positions"
  misc_feature 1..732: note = source = /note="Description of Artificial Sequence: Synthetic polynucleotide"
  misc_feature 1..732: note = source = /note="See specification as filed for detailed description of substitutions and preferred embodiments"
  source 1..732: mol_type = other DNA
caggtgaccctgagagagagcggccccgccctggtgaagcccacccagaccctgaccctgacctgcaccgtgagcggcttcagcctgaccagctacagcgtgcactgggtgagacagccccccggcaagggcctggagtggctgggcgtgatctgggccagcggcggcaccgactacaacagcgccctgatgagcagactgagcatcagcaaggacaccagcagaaaccaggtggtgctgaccatgaccaacatggaccccgtggacaccgccacctactactgcgccagagacccccccagcagcctgctgagactggactactggggcagaggcacccccgtgaccgtgagcagcgccagcaccaagggccccagcgtgttccccctggcccccagcagcaagagcaccagcggcggcaccgccgccctgggctgcctggtgaaggactacttccccgagcccgtgaccgtgagctggaacagcggcgccctgaccagcggcgtgcacaccttccccgccgtgctgcagagcagcggcctgtacagcctgagcagcgtggtgaccgtgcccagcagcagcctgggcacccagacctacatctgcaacgtgaaccacaagcccagcaacaccaaggtggacaagagagtggagcccaagagctgcgacaagacccacacctgccccccctgccccgcccccgagctgctgggcggccccagcgtgttcctg

SEQ ID NO: 116 - DNA, 657 bp, synthetic construct
  misc_feature 1..657: note = source = /note="Description of Artificial Sequence: Synthetic polynucleotide"
  source 1..657: mol_type = other DNA
gacatcgtgatgacccagagccccgacagcctggccgtgagcctgggcgagagagccaccatcaactgcaagagcagccagagcctgctgaacagcggcaaccagaagaactacctggcctggcagcagaagcccggccagccccccaagctgctgatctacggcgccagcaccagagagagcggcgtgcccgacagattcagcggcagcggcagcggcaccgacttcaccctgaccatcagcagcctgcaggccgaggacgtggccgtgtactactgccagaacgtgcacagcttccccttcaccttcggcggcggcaccaagctggagatcaagagaaccgtggccgcccccagcgtgttcatcttcccccccagcgacgagcagctgaagagcggcaccgccagcgtggtgtgcctgctgaacaacttctaccccagagaggccaaggtgcagtggaaggtggacaacgccctgcagagcggcaacagccaggagagcgtgaccgagcaggacagcaaggacagcacctacagcctgagcagcaccctgaccctgagcaaggccgactacgagaagcacaaggtgtacgcctgcgaggtgacccaccagggcctgagcagccccgtgaccaagagcttcaacagaggcgagtgc

SEQ ID NO: 117 - DNA, 738 bp, synthetic construct
  misc_feature 676..738: note = /note="This region may be absent in its entirety"
  variation 685..687: replace = ctg
  misc_feature 688..738: note = /note="This region may be absent in its entirety"
  misc_feature 706..738: note = /note="This region may be absent in its entirety"
  misc_feature 1..738: note = /note="Variant nucleotides given in the sequence have no preference with respect to those in the annotations for variant positions"
  misc_feature 1..738: note = source = /note="Description of Artificial Sequence: Synthetic polynucleotide"
  misc_feature 1..738: note = source = /note="See specification as filed for detailed description of substitutions and preferred embodiments"
  source 1..738: mol_type = other DNA
caggtgcagctggtgcagagcggcgccgaggtgaagaagcccggcgccagcgtgaaggtgagctgcaagggcagcggctacaccttcaccagctactggatgcactgggtgagacaggcccccggccagagactggagtggatcggcgagatcgaccccagcgagagcaacaccaactacaaccagaagttcaagggcagagtgaccctgaccgtggacatcagcgccagcaccgcctacatggagctgagcagcctgagaagcgaggacaccgccgtgtactactgcgccagaggcggctacgacggctgggactacgccatcgactactggggccagggcaccctggtgaccgtgagcagcgccagcaccaagggccccagcgtgttccccctggcccccagcagcaagagcaccagcggcggcaccgccgccctgggctgcctggtgaaggactacttccccgagcccgtgaccgtgagctggaacagcggcgccctgaccagcggcgtgcacaccttccccgccgtgctgcagagcagcggcctgtacagcctgagcagcgtggtgaccgtgcccagcagcagcctgggcacccagacctacatctgcaacgtgaaccacaagcccagcaacaccaaggtggacaagaaggtggagcccaagagctgcgacaagacccacacctgccccccctgccccgcccccgagctggccggcgcccccagcgtgttcctg

SEQ ID NO: 118 - DNA, 657 bp, synthetic construct
  misc_feature 1..657: note = source = /note="Description of Artificial Sequence: Synthetic polynucleotide"
  source 1..657: mol_type = other DNA
gacgtggtgatgacccagagccccctgagcctgcccgtgacccccggcgagcccgccagcatcagctgcagaagcagccagagcctggccaagagctacggcaacacctacctgagctggtacctgcagaagcccggccagagcccccagctgctgatctacggcatcagcaacagattcagcggcgtgcccgacagattcagcggcagcggcagcggcaccgacttcaccctgaagatcagcagagtggaggccgaggacgtgggcgtgtactactgcctgcagggcacccaccagccctacaccttcggccagggcaccaaggtggagatcaagagaaccgtggccgcccccagcgtgttcatcttcccccccagcgacgagcagctgaagagcggcaccgccagcgtggtgtgcctgctgaacaacttctaccccagagaggccaaggtgcagtggaaggtggacaacgccctgcagagcggcaacagccaggagagcgtgaccgagcaggacagcaaggacagcacctacagcctgagcagcaccctgaccctgagcaaggccgactacgagaagcacaaggtgtacgcctgcgaggtgacccaccagggcctgagcagccccgtgaccaagagcttcaacagaggcgagtgc

SEQ ID NO: 119 - DNA, 735 bp, synthetic construct
  misc_feature 676..735: note = /note="This region may be absent in its entirety"
  misc_feature 703..735: note = /note="This region may be absent in its entirety"
  misc_feature 1..735: note = source = /note="Description of Artificial Sequence: Synthetic polynucleotide"
  misc_feature 1..735: note = source = /note="See specification as filed for detailed description of substitutions and preferred embodiments"
  source 1..735: mol_type = other DNA
caggtgcagctggtgcagagcggcgccgaggtgaagaagcccggcgccagcgtgaaggtgagctgcaaggccagcggcttcaacatcaaggacacctacatccactgggtgagacaggcccccggccagagactggagtggatgggcagaatcgaccccgccaacggctacaccaagtacgaccccaagttccagggcagagtgaccatcaccgccgacaccagcgccagcaccgcctacatggagctgagcagcctgagaagcgaggacaccgccgtgtactactgcgccagagagggctactacggcaactacggcgtgtacgccatggactactggggccagggcaccctggtgaccgtgagcagcgccagcaccaagggccccagcgtgttccccctggccccctgcagcagaagcaccagcgagagcaccgccgccctgggctgcctggtgaaggactacttccccgagcccgtgaccgtgagctggaacagcggcgccctgaccagcggcgtgcacaccttccccgccgtgctgcagagcagcggcctgtacagcctgagcagcgtggtgaccgtgcccagcagcagcctgggcaccaagacctacacctgcaacgtggaccacaagcccagcaacaccaaggtggacaagagagtggagagcaagtacggccccccctgccccccctgccccgcccccgagttcctgggcggccccagcgtgttcctg

SEQ ID NO: 120 - DNA, 639 bp, synthetic construct
  misc_feature 1..639: note = source = /note="Description of Artificial Sequence: Synthetic polynucleotide"
  source 1..639: mol_type = other DNA
gacatccagatgacccagagccccagcagcctgagcgccagcgtgggcgacagagtgaccatcacctgcaagaccagccaggacatcaacaagtacatggcctggtaccagcagacccccggcaaggcccccagactgctgatccactacaccagcgccctgcagcccggcatccccagcagattcagcggcagcggcagcggcagagactacaccttcaccatcagcagcctgcagcccgaggacatcgccacctactactgcctgcagtacgacaacctgtggaccttcggccagggcaccaaggtggagatcaagagaaccgtggccgcccccagcgtgttcatcttcccccccagcgacgagcagctgaagagcggcaccgccagcgtggtgtgcctgctgaacaacttctaccccagagaggccaaggtgcagtggaaggtggacaacgccctgcagagcggcaacagccaggagagcgtgaccgagcaggacagcaaggacagcacctacagcctgagcagcaccctgaccctgagcaaggccgactacgagaagcacaaggtgtacgcctgcgaggtgacccaccagggcctgagcagccccgtgaccaagagcttcaacagaggcgagtgc

SEQ ID NO: 121 - DNA, 729 bp, synthetic construct
  misc_feature 667..729: note = /note="This region may be absent in its entirety"
  variation 676..678: replace = ctg
  misc_feature 679..729: note = /note="This region may be absent in its entirety"
  misc_feature 697..729: note = /note="This region may be absent in its entirety"
  misc_feature 1..729: note = /note="Variant nucleotides given in the sequence have no preference with respect to those in the annotations for variant positions"
  misc_feature 1..729: note = source = /note="Description of Artificial Sequence: Synthetic polynucleotide"
  misc_feature 1..729: note = source = /note="See specification as filed for detailed description of substitutions and preferred embodiments"
  source 1..729: mol_type = other DNA
gaggtgcagctggtggagagcggcggcggcctggtgcagcccggcggcagcctgagactgagctgcgccgccagcggcttcaccttcaacaactacgccatgaactgggtgagacaggcccccggcaagggcctggactgggtgagcaccatcagcggcagcggcggcaccaccaactacgccgacagcgtgaagggcagattcatcatcagcagagacagcagcaagcacaccctgtacctgcagatgaacagcctgagagccgaggacaccgccgtgtactactgcgccaaggacagcaactggggcaacttcgacctgtggggcagaggcaccctggtgaccgtgagcagcgccagcaccaagggccccagcgtgttccccctggcccccagcagcaagagcaccagcggcggcaccgccgccctgggctgcctggtgaaggactacttccccgagcccgtgaccgtgagctggaacagcggcgccctgaccagcggcgtgcacaccttccccgccgtgctgcagagcagcggcctgtacagcctgagcagcgtggtgaccgtgcccagcagcagcctgggcacccagacctacatctgcaacgtgaaccacaagcccagcaacaccaaggtggacaagaaggtggagcccaagagctgcgacaagacccacacctgccccccctgccccgcccccgagctgctgggcggccccagcgtgttcctg

SEQ ID NO: 122 - DNA, 660 bp, synthetic construct
  misc_feature 1..660: note = source = /note="Description of Artificial Sequence: Synthetic polynucleotide"
  source 1..660: mol_type = other DNA
gacatcgtgatgacccagagccccgacagcctggccgtgagcctgggcgagagagccaccatcaactgcaagagcagccagagcgtgctgtacagaagcaacaacagaaacttcctgggctggtaccagcagaagcccggccagccccccaacctgctgatctactgggccagcaccagagagagcggcgtgcccgacagattcagcggcagcggcagcggcaccgacttcaccctgaccatcagcagcctgcaggccgaggacgtggccgtgtactactgccagcagtactacaccaccccctacaccttcggccagggcaccaagctggagatcaagagaaccgtggccgcccccagcgtgttcatcttcccccccagcgacgagcagctgaagagcggcaccgccagcgtggtgtgcctgctgaacaacttctaccccagagaggccaaggtgcagtggaaggtggacaacgccctgcagagcggcaacagccaggagagcgtgaccgagcaggacagcaaggacagcacctacagcctgagcagcaccctgaccctgagcaaggccgactacgagaagcacaaggtgtacgcctgcgaggtgacccaccagggcctgagcagccccgtgaccaagagcttcaacagaggcgagtgc

SEQ ID NO: 123 - DNA, 693 bp, synthetic construct
  misc_feature 661..693: note = /note="This region may be absent in its entirety"
  misc_feature 679..693: note = /note="This region may be absent in its entirety"
  misc_feature 1..693: note = source = /note="Description of Artificial Sequence: Synthetic polynucleotide"
  misc_feature 1..693: note = source = /note="See specification as filed for detailed description of substitutions and preferred embodiments"
  source 1..693: mol_type = other DNA
gaggtgcagctggtgcagagcggcgccgaggtgaagaagcccggcgccagcgtgaaggtgagctgcaaggccagcggctacaccctgaccagctacggcatcagctgggtgagacaggcccccggccagggcctggagtggatgggctgggtgagcttctacaacggcaacaccaactacgcccagaagctgcagggcagaggcaccatgaccaccgaccccagcaccagcaccgcctacatggagctgagaagcctgagaagcgacgacaccgccgtgtactactgcgccagaggctacggcatggacgtgtggggccagggcaccaccgtgaccgtgagcagcgccagcaccaagggccccagcgtgttccccctggccccctgcagcagaagcaccagcgagagcaccgccgccctgggctgcctggtgaaggactacttccccgagcccgtgaccgtgagctggaacagcggcgccctgaccagcggcgtgcacaccttccccgccgtgctgcagagcagcggcctgtacagcctgagcagcgtggtgaccgtgcccagcagcaacttcggcacccagacctacacctgcaacgtggaccacaagcccagcaacaccaaggtggacaagaccgtggagagaaagtgctgcgtggagtgccccccctgccccgccccccccgtggccggc

SEQ ID NO: 124 - DNA, 645 bp, synthetic construct
  misc_feature 1..645: note = source = /note="Description of Artificial Sequence: Synthetic polynucleotide"
  source 1..645: mol_type = other DNA
gagagcgccctgacccagcccgccagcgtgagcggcagccccggccagagcatcaccatcagctgcaccggcaccagcagcgacgtgggcggctacaacagcgtgagctggtaccagcagcaccccggcaaggcccccaagctgatgatctacgaggtgagcaacagacccagcggcgtgagcaacagattcagcggcagcaagagcggcaacaccgccagcctgaccatcagcggcctgcaggccgaggacgaggccgactactactgcaacagctacaccagcaccagcatggtgttcggcggcggcaccaagctgaccgtgctgggccagcccaaggccgcccccagcgtgaccctgttcccccccagcagcgaggagctgcaggccaacaaggccaccctggtgtgcctgatcagcgacttctaccccggcgccgtgaccgtggcctggaaggccgacagcagccccgtgaaggccggcgtggagaccaccacccccagcaagcagagcaacaacaagtacgccgccagcagctacctgagcctgacccccgagcagtggaagagccacagaagctacagctgccaggtgacccacgagggcagcaccgtggagaagaccgtggcccccaccgagtgcagc

SEQ ID NO: 125 - DNA, 744 bp, synthetic construct
  misc_feature 694..744: note = /note="This region may be absent in its entirety"
  misc_feature 712..744: note = /note="This region may be absent in its entirety"
  misc_feature 1..744: note = source = /note="Description of Artificial Sequence: Synthetic polynucleotide"
  misc_feature 1..744: note = source = /note="See specification as filed for detailed description of substitutions and preferred embodiments"
  source 1..744: mol_type = other DNA
gaggtgcagctggtggagagcggcggcggcgtgatccagcccggcggcagcctgagactgagctgcgccgccagcggcttcaccttcgacgactacgccatgaactgggtgagacagggccccggcaagggcctggagtgggtgagcgccatcagcggcgacggcggcagcacctactacgccgacagcgtgaagggcagattcaccatcagcagagacaacagcaagaacagcctgtacctgcagatgaacagcctgagagccgaggacaccgccttcttctactgcgccaaggacctgagaaacaccatcttcggcgtggtgatccccgacgccttcgacatctggggccagggcaccatggtgaccgtgagcagcgccagcaccaagggccccagcgtgttccccctggccccctgcagcagaagcaccagcgagagcaccgccgccctgggctgcctggtgaaggactacttccccgagcccgtgaccgtgagctggaacagcggcgccctgaccagcggcgtgcacaccttccccgccgtgctgcagagcagcggcctgtacagcctgagcagcgtggtgaccgtgcccagcagcagcctgggcaccaagacctacacctgcaacgtggaccacaagcccagcaacaccaaggtggacaagagagtggagagcaagtacggccccccctgccccccctgccccgcccccgagttcctgggcggccccagcgtgttcctg

SEQ ID NO: 126 - DNA, 642 bp, synthetic construct
  misc_feature 1..642: note = source = /note="Description of Artificial Sequence: Synthetic polynucleotide"
  source 1..642: mol_type = other DNA
gacatccagatgacccagagccccagcaccctgagcgccagcgtgggcgacagagtgaccatcacctgcagagccagccagagcatcagaagctggctggcctggtaccagcagaagcccggcaaggcccccaagctgctgatctacaaggccagcagcctggagagcggcgtgcccagcagattcagcggcagcggcagcggcaccgagttcaccctgaccatcagcagcctgcagcccgacgacttcgccacctactactgccagcagtacaacagctacagctacaccttcggccagggcaccaagctggagatcaagagaaccgtggccgcccccagcgtgttcatcttcccccccagcgacgagcagctgaagagcggcaccgccagcgtggtgtgcctgctgaacaacttctaccccagagaggccaaggtgcagtggaaggtggacaacgccctgcagagcggcaacagccaggagagcgtgaccgagcaggacagcaaggacagcacctacagcctgagcagcaccctgaccctgagcaaggccgactacgagaagcacaaggtgtacgcctgcgaggtgacccaccagggcctgagcagccccgtgaccaagagcttcaacagaggcgagtgc

SEQ ID NO: 127 - DNA, 741 bp, synthetic construct
  misc_feature 679..741: note = /note="This region may be absent in its entirety"
  variation 688..690: replace = ctg
  misc_feature 691..741: note = /note="This region may be absent in its entirety"
  misc_feature 709..741: note = /note="This region may be absent in its entirety"
  misc_feature 1..741: note = /note="Variant nucleotides given in the sequence have no preference with respect to those in the annotations for variant positions"
  misc_feature 1..741: note = source = /note="Description of Artificial Sequence: Synthetic polynucleotide"
  misc_feature 1..741: note = source = /note="See specification as filed for detailed description of substitutions and preferred embodiments"
  source 1..741: mol_type = other DNA
gaggtgcagctgctggagagcggcggcggcctggtgcagcccggcggcagcctgagactgagctgcgccgccagcggcttcaccttcagcagctacgccatgagctgggtgagacaggcccccggcaagggcctggagtgggtgagcggcatcaccggcagcggcggcagcacctactacgccgacagcgtgaagggcagattcaccatcagcagagacaacagcaagaacaccctgtacctgcagatgaacagcctgagagccgaggacaccgccgtgtactactgcgccaaggaccccggcaccaccgtgatcatgagctggttcgacccctggggccagggcaccctggtgaccgtgagcagcgccagcaccaagggccccagcgtgttccccctggcccccagcagcaagagcaccagcggcggcaccgccgccctgggctgcctggtgaaggactacttccccgagcccgtgaccgtgagctggaacagcggcgccctgaccagcggcgtgcacaccttccccgccgtgctgcagagcagcggcctgtacagcctgagcagcgtggtgaccgtgcccagcagcagcctgggcacccagacctacatctgcaacgtgaaccacaagcccagcaacaccaaggtggacaagaaggtggagcccaagagctgcgacaagacccacacctgccccccctgccccgcccccgagctgctgggcggccccagcgtgttcctg

SEQ ID NO: 128 - DNA, 645 bp, synthetic construct
  misc_feature 1..645: note = source = /note="Description of Artificial Sequence: Synthetic polynucleotide"
  source 1..645: mol_type = other DNA
gagatcgtgctgacccagagccccggcaccctgagcctgagccccggcgagagagccaccctgagctgcagagccagccagagcgtgagaggcagatacctggcctggtaccagcagaagcccggccaggcccccagactgctgatctacggcgccagcagcagagccaccggcatccccgacagattcagcggcagcggcagcggcaccgacttcaccctgaccatcagcagactggagcccgaggacttcgccgtgttctactgccagcagtacggcagcagccccagaaccttcggccagggcaccaaggtggagatcaagagaaccgtggccgcccccagcgtgttcatcttcccccccagcgacgagcagctgaagagcggcaccgccagcgtggtgtgcctgctgaacaacttctaccccagagaggccaaggtgcagtggaaggtggacaacgccctgcagagcggcaacagccaggagagcgtgaccgagcaggacagcaaggacagcacctacagcctgagcagcaccctgaccctgagcaaggccgactacgagaagcacaaggtgtacgcctgcgaggtgacccaccagggcctgagcagccccgtgaccaagagcttcaacagaggcgagtgc

SEQ ID NO: 129 - DNA, 705 bp, synthetic construct
  misc_feature 646..705: note = /note="This region may be absent in its entirety"
  misc_feature 673..705: note = /note="This region may be absent in its entirety"
  misc_feature 1..705: note = source = /note="Description of Artificial Sequence: Synthetic polynucleotide"
  misc_feature 1..705: note = source = /note="See specification as filed for detailed description of substitutions and preferred embodiments"
  source 1..705: mol_type = other DNA
caggtgcagctggtggagagcggcggcggcgtggtgcagcccggcagaagcctgagactggactgcaaggccagcggcatcaccttcagcaacagcggcatgcactgggtgagacaggcccccggcaagggcctggagtgggtggccgtgatctggtacgacggcagcaagagatactacgccgacagcgtgaagggcagattcaccatcagcagagacaacagcaagaacaccctgttcctgcagatgaacagcctgagagccgaggacaccgccgtgtactactgcgccaccaacgacgactactggggccagggcaccctggtgaccgtgagcagcgccagcaccaagggccccagcgtgttccccctggccccctgcagcagaagcaccagcgagagcaccgccgccctgggctgcctggtgaaggactacttccccgagcccgtgaccgtgagctggaacagcggcgccctgaccagcggcgtgcacaccttccccgccgtgctgcagagcagcggcctgtacagcctgagcagcgtggtgaccgtgcccagcagcagcctgggcaccaagacctacacctgcaacgtggaccacaagcccagcaacaccaaggtggacaagagagtggagagcaagtacggccccccctgccccccctgccccgcccccgagttcctgggcggccccagcgtgttcctg

SEQ ID NO: 130 - DNA, 642 bp, synthetic construct
  misc_feature 1..642: note = source = /note="Description of Artificial Sequence: Synthetic polynucleotide"
  source 1..642: mol_type = other DNA
gagatcgtgctgacccagagccccgccaccctgagcctgagccccggcgagagagccaccctgagctgcagagccagccagagcgtgagcagctacctggcctggtaccagcagaagcccggccaggcccccagactgctgatctacgacgccagcaacagagccaccggcatccccgccagattcagcggcagcggcagcggcaccgacttcaccctgaccatcagcagcctggagcccgaggacttcgccgtgtactactgccagcagagcagcaactggcccagaaccttcggccagggcaccaaggtggagatcaagagaaccgtggccgcccccagcgtgttcatcttcccccccagcgacgagcagctgaagagcggcaccgccagcgtggtgtgcctgctgaacaacttctaccccagagaggccaaggtgcagtggaaggtggacaacgccctgcagagcggcaacagccaggagagcgtgaccgagcaggacagcaaggacagcacctacagcctgagcagcaccctgaccctgagcaaggccgactacgagaagcacaaggtgtacgcctgcgaggtgacccaccagggcctgagcagccccgtgaccaagagcttcaacagaggcgagtgc

SEQ ID NO: 131 - DNA, 726 bp, synthetic construct
  misc_feature 667..726: note = /note="This region may be absent in its entirety"
  misc_feature 694..726: note = /note="This region may be absent in its entirety"
  misc_feature 1..726: note = source = /note="Description of Artificial Sequence: Synthetic polynucleotide"
  misc_feature 1..726: note = source = /note="See specification as filed for detailed description of substitutions and preferred embodiments"
  source 1..726: mol_type = other DNA
caggtgcagctggtgcagagcggcgtggaggtgaagaagcccggcgccagcgtgaaggtgagctgcaaggccagcggctacaccttcaccaactactacatgtactgggtgagacaggcccccggccagggcctggagtggatgggcggcatcaaccccagcaacggcggcaccaacttcaacgagaagttcaagaacagagtgaccctgaccaccgacagcagcaccaccaccgcctacatggagctgaagagcctgcagttcgacgacaccgccgtgtactactgcgccagaagagactacagattcgacatgggcttcgactactggggccagggcaccaccgtgaccgtgagcagcgccagcaccaagggccccagcgtgttccccctggccccctgcagcagaagcaccagcgagagcaccgccgccctgggctgcctggtgaaggactacttccccgagcccgtgaccgtgagctggaacagcggcgccctgaccagcggcgtgcacaccttccccgccgtgctgcagagcagcggcctgtacagcctgagcagcgtggtgaccgtgcccagcagcagcctgggcaccaagacctacacctgcaacgtggaccacaagcccagcaacaccaaggtggacaagagagtggagagcaagtacggccccccctgccccccctgccccgcccccgagttcctgggcggccccagcgtgttcctg

SEQ ID NO: 132 - DNA, 654 bp, synthetic construct
  misc_feature 1..654: note = source = /note="Description of Artificial Sequence: Synthetic polynucleotide"
  source 1..654: mol_type = other DNA
gagatcgtgctgacccagagccccgccaccctgagcctgagccccggcgagagagccaccctgagctgcagagccagcaagggcgtgagcaccagcggctacagctacctgcactggtaccagcagaagcccggccaggcccccagactgctgatctacctggccagctacctggagagcggcgtgcccgccagattcagcggcagcggcagcggcaccgacttcaccctgaccatcagcagcctggagcccgaggacttcgccgtgtactactgccagcacagcagagacctgcccctgaccttcggcggcggcaccaaggtggagatcaagagaaccgtggccgcccccagcgtgttcatcttcccccccagcgacgagcagctgaagagcggcaccgccagcgtggtgtgcctgctgaacaacttctaccccagagaggccaaggtgcagtggaaggtggacaacgccctgcagagcggcaacagccaggagagcgtgaccgagcaggacagcaaggacagcacctacagcctgagcagcaccctgaccctgagcaaggccgactacgagaagcacaaggtgtacgcctgcgaggtgacccaccagggcctgagcagccccgtgaccaagagcttcaacagaggcgagtgc

SEQ ID NO: 133 - DNA, 744 bp, synthetic construct
  misc_feature 682..744: note = /note="This region may be absent in its entirety"
  variation 691..693: replace = ctg
  misc_feature 694..744: note = /note="This region may be absent in its entirety"
  misc_feature 712..744: note = /note="This region may be absent in its entirety"
  misc_feature 1..744: note = /note="Variant nucleotides given in the sequence have no preference with respect to those in the annotations for variant positions"
  misc_feature 1..744: note = source = /note="Description of Artificial Sequence: Synthetic polynucleotide"
  misc_feature 1..744: note = source = /note="See specification as filed for detailed description of substitutions and preferred embodiments"
  source 1..744: mol_type = other DNA
gaggtgcagctggtggagagcggcggcggcctggtgcagcccggcggcagcctgagactgagctgcgccgccagcggctacgacttcacccactacggcatgaactgggtgagacaggcccccggcaagggcctggagtgggtgggctggatcaacacctacaccggcgagcccacctacgccgccgacttcaagagaagattcaccttcagcctggacaccagcaagagcaccgcctacctgcagatgaacagcctgagagccgaggacaccgccgtgtactactgcgccaagtacccctactactacggcaccagccactggtacttcgacgtgtggggccagggcaccctggtgaccgtgagcagcgccagcaccaagggccccagcgtgttccccctggcccccagcagcaagagcaccagcggcggcaccgccgccctgggctgcctggtgaaggactacttccccgagcccgtgaccgtgagctggaacagcggcgccctgaccagcggcgtgcacaccttccccgccgtgctgcagagcagcggcctgtacagcctgagcagcgtggtgaccgtgcccagcagcagcctgggcacccagacctacatctgcaacgtgaaccacaagcccagcaacaccaaggtggacaagaaggtggagcccaagagctgcgacaagacccacacctgccccccctgccccgcccccgagctgctgggcggccccagcgtgttcctg

SEQ ID NO: 134 - DNA, 642 bp, synthetic construct
  misc_feature 1..642: note = source = /note="Description of Artificial Sequence: Synthetic polynucleotide"
  source 1..642: mol_type = other DNA
gacatccagctgacccagagccccagcagcctgagcgccagcgtgggcgacagagtgaccatcacctgcagcgccagccaggacatcagcaactacctgaactggtaccagcagaagcccggcaaggcccccaaggtgctgatctacttcaccagcagcctgcacagcggcgtgcccagcagattcagcggcagcggcagcggcaccgacttcaccctgaccatcagcagcctgcagcccgaggacttcgccacctactactgccagcagtacagcaccgtgccctggaccttcggccagggcaccaaggtggagatcaagagaaccgtggccgcccccagcgtgttcatcttcccccccagcgacgagcagctgaagagcggcaccgccagcgtggtgtgcctgctgaacaacttctaccccagagaggccaaggtgcagtggaaggtggacaacgccctgcagagcggcaacagccaggagagcgtgaccgagcaggacagcaaggacagcacctacagcctgagcagcaccctgaccctgagcaaggccgactacgagaagcacaaggtgtacgcctgcgaggtgacccaccagggcctgagcagccccgtgaccaagagcttcaacagaggcgagtgc

SEQ ID NO: 135 - DNA, 744 bp, synthetic construct
  misc_feature 682..744: note = /note="This region may be absent in its entirety"
  variation 691..693: replace = ctg
  misc_feature 694..744: note = /note="This region may be absent in its entirety"
  misc_feature 712..744: note = /note="This region may be absent in its entirety"
  misc_feature 1..744: note = /note="Variant nucleotides given in the sequence have no preference with respect to those in the annotations for variant positions"
  misc_feature 1..744: note = source = /note="Description of Artificial Sequence: Synthetic polynucleotide"
  misc_feature 1..744: note = source = /note="See specification as filed for detailed description of substitutions and preferred embodiments"
  source 1..744: mol_type = other DNA
gaggtgcagctggtggagagcggcggcggcctggtgcagcccggcggcagcctgagactgagctgcgccgccagcggctacaccttcaccaactacggcatgaactgggtgagacaggcccccggcaagggcctggagtgggtgggctggatcaacacctacaccggcgagcccacctacgccgccgacttcaagagaagattcaccttcagcctggacaccagcaagagcaccgcctacctgcagatgaacagcctgagagccgaggacaccgccgtgtactactgcgccaagtacccccactactacggcagcagccactggtacttcgacgtgtggggccagggcaccctggtgaccgtgagcagcgccagcaccaagggccccagcgtgttccccctggcccccagcagcaagagcaccagcggcggcaccgccgccctgggctgcctggtgaaggactacttccccgagcccgtgaccgtgagctggaacagcggcgccctgaccagcggcgtgcacaccttccccgccgtgctgcagagcagcggcctgtacagcctgagcagcgtggtgaccgtgcccagcagcagcctgggcacccagacctacatctgcaacgtgaaccacaagcccagcaacaccaaggtggacaagaaggtggagcccaagagctgcgacaagacccacacctgccccccctgccccgcccccgagctgctgggcggccccagcgtgttcctg

SEQ ID NO: 136 - DNA, 642 bp, synthetic construct
  misc_feature 1..642: note = source = /note="Description of Artificial Sequence: Synthetic polynucleotide"
  source 1..642: mol_type = other DNA
gacatccagatgacccagagccccagcagcctgagcgccagcgtgggcgacagagtgaccatcacctgcagcgccagccaggacatcagcaactacctgaactggtaccagcagaagcccggcaaggcccccaaggtgctgatctacttcaccagcagcctgcacagcggcgtgcccagcagattcagcggcagcggcagcggcaccgacttcaccctgaccatcagcagcctgcagcccgaggacttcgccacctactactgccagcagtacagcaccgtgccctggaccttcggccagggcaccaaggtggagatcaagagaaccgtggccgcccccagcgtgttcatcttcccccccagcgacgagcagctgaagagcggcaccgccagcgtggtgtgcctgctgaacaacttctaccccagagaggccaaggtgcagtggaaggtggacaacgccctgcagagcggcaacagccaggagagcgtgaccgagcaggacagcaaggacagcacctacagcctgagcagcaccctgaccctgagcaaggccgactacgagaagcacaaggtgtacgcctgcgaggtgacccaccagggcctgagcagccccgtgaccaagagcttcaacagaggcgagtgc

SEQ ID NO: 137 - DNA, 720 bp, synthetic construct
  misc_feature 658..720: note = /note="This region may be absent in its entirety"
  variation 667..669: replace = ctg
  misc_feature 670..720: note = /note="This region may be absent in its entirety"
  misc_feature 688..720: note = /note="This region may be absent in its entirety"
  misc_feature 1..720: note = /note="Variant nucleotides given in the sequence have no preference with respect to those in the annotations for variant positions"
  misc_feature 1..720: note = source = /note="Description of Artificial Sequence: Synthetic polynucleotide"
  misc_feature 1..720: note = source = /note="See specification as filed for detailed description of substitutions and preferred embodiments"
  source 1..720: mol_type = other DNA
gaggtgcagctggtgcagagcggccccgagctgaagaagcccggcgccagcgtgaaggtgagctgcaaggccagcggctacaccttcaccaactacggcatgaactgggtgagacaggcccccggccagggcctggagtggatgggctggatcaacacctacaccggcgagaccacctacgccgacgacttcaagggcagattcgtgttcagcctggacaccagcgtgagcaccgcctacctgcagatcagcagcctgaaggccgaggacaccgccgtgtactactgcgagagagagggcggcgtgaacaactggggccagggcaccctggtgaccgtgagcagcgccagcaccaagggccccagcgtgttccccctggcccccagcagcaagagcaccagcggcggcaccgccgccctgggctgcctggtgaaggactacttccccgagcccgtgaccgtgagctggaacagcggcgccctgaccagcggcgtgcacaccttccccgccgtgctgcagagcagcggcctgtacagcctgagcagcgtggtgaccgtgcccagcagcagcctgggcacccagacctacatctgcaacgtgaaccacaagcccagcaacaccaaggtggacaagaaggtggagcccaagagctgcgacaagacccacacctgccccccctgccccgcccccgagctgctgggcggccccagcgtgttcctg

SEQ ID NO: 138 - DNA, 642 bp, synthetic construct
  misc_feature 1..642: note = source = /note="Description of Artificial Sequence: Synthetic polynucleotide"
  source 1..642: mol_type = other DNA
gacatccaggtgacccagagccccagcagcctgagcgccagcgtgggcgacagagtgaccatcacctgcatcaccagcaccgacatcgacgacgacatgaactggtaccagcagaagcccggcaaggtgcccaagctgctgatcagcggcggcaacaccctgagacccggcgtgcccagcagattcagcggcagcggcagcggcaccgacttcaccctgaccatcagcagcctgcagcccgaggacgtggccacctactactgcctgcagagcgacagcctgccctacaccttcggccagggcaccaaggtggagatcaagagaaccgtggccgcccccagcgtgttcatcttcccccccagcgacgagcagctgaagagcggcaccgccagcgtggtgtgcctgctgaacaacttctaccccagagaggccaaggtgcagtggaaggtggacaacgccctgcagagcggcaacagccaggagagcgtgaccgagcaggacagcaaggacagcacctacagcctgagcagcaccctgaccctgagcaaggccgactacgagaagcacaaggtgtacgcctgcgaggtgacccaccagggcctgagcagccccgtgaccaagagcttcaacagaggcgagtgc

SEQ ID NO: 139 - DNA, 360 bp, synthetic construct
  misc_feature 1..360: note = source = /note="Description of Artificial Sequence: Synthetic polynucleotide"
  source 1..360: mol_type = other DNA
gaggtgcagctggtggagagcggcggcggcctggtgcagcccggcggcagcctgagactgagctgcaccgccagcggcttcagcctgaccgactactactacatgacctgggtgagacaggcccccggcaagggcctggagtgggtgggcttcatcgaccccgacgacgacccctactacgccacctgggccaagggcagattcaccatcagcagagacaacagcaagaacaccctgtacctgcagatgaacagcctgagagccgaggacaccgccgtgtactactgcgccggcggcgaccacaacagcggctggggcctggacatctggggccagggcaccctggtgaccgtgagcagc

SEQ ID NO: 140 - DNA, 333 bp, synthetic construct
  misc_feature 1..333: note = source = /note="Description of Artificial Sequence: Synthetic polynucleotide"
  source 1..333: mol_type = other DNA
gagatcgtgatgacccagagccccagcaccctgagcgccagcgtgggcgacagagtgatcatcacctgccaggccagcgagatcatccacagctggctggcctggtaccagcagaagcccggcaaggcccccaagctgctgatctacctggccagcaccctggccagcggcgtgcccagcagattcagcggcagcggcagcggcgccgagttcaccctgaccatcagcagcctgcagcccgacgacttcgccacctactactgccagaacgtgtacctggccagcaccaacggcgccaacttcggccagggcaccaagctgaccgtgctgggc

SEQ ID NO: 141 - DNA, 741 bp, synthetic construct
  misc_feature 679..741: note = /note="This region may be absent in its entirety"
  variation 688..690: replace = ctg
  misc_feature 691..741: note = /note="This region may be absent in its entirety"
  misc_feature 709..741: note = /note="This region may be absent in its entirety"
  misc_feature 1..741: note = /note="Variant nucleotides given in the sequence have no preference with respect to those in the annotations for variant positions"
  misc_feature 1..741: note = source = /note="Description of Artificial Sequence: Synthetic polynucleotide"
  misc_feature 1..741: note = source = /note="See specification as filed for detailed description of substitutions and preferred embodiments"
  source 1..741: mol_type = other DNA
caggtgcagctgcagcagagcggcgcggaagtgaaaaaaccgggcagcagcgtgcgcgtgagctgcaaagcgagcggcggcacctttaacaacaacgcgattaactgggtgcgccaggcgccgggccagggcctggaatggatgggcggcattattccgatgtttggcaccgcgaaatatagccagaactttcagggccgcgtggcgattaccgcggatgaaagcaccggcaccgcgagcatggaactgagcagcctgcgcagcgaagataccgcggtgtattattgcgcgcgcagccgcgatctgctgctgtttccgcatcatgcgctgagcccgtggggccgcggcaccatggtgaccgtgagcagcgcgagcaccaaaggcccgagcgtgtttccgctggcgccgagcagcaaaagcaccagcggcggcaccgcggcgctgggctgcctggtgaaagattattttccggaaccggtgaccgtgagcaacagcggcgcgctgaccagcggcgtgcatacctttccggcggtgctgcagagcagcggcctgtatagcctgagcagcgtggtgaccgtgccgagcagcagcctgggcacccagacctatatttgcaacgtgaaccataaaccgagcaacaccaaagtggataaaaaagtggaaccgaaaagctgcgataaaacccatacctgcccgccgtgcccggcgccggaactgctgggcggcccgagcgtgtttctg

SEQ ID NO: 142 - DNA, 639 bp, synthetic construct
  misc_feature 1..639: note = source = /note="Description of Artificial Sequence: Synthetic polynucleotide"
  source 1..639: mol_type = other DNA
agcagcgaactgacccaggatccggcggtgagcgtggcgctgggccagaccgtgcgcgtgacctgccagggcgatagcctgcgcagctattatgcgagctggtatcagcagaaaccgggccaggcgccggtgctggtgatttatggcaaaaacaaccgcccgagcggcattccggatcgctttagcggcagcagcagcggcaacaccgcgagcctgaccattaccggcgcgcaggcggaagatgaagcggattattattgcagcagccgcgatagcagcggcaaccattgggtgtttggcggcggcaccgaactgaccgtgctgggccagccgaaagcggcgccgagcgtgaccctgtttccgccgagcagcgaagaactgcaggcgaacaaagcgaccctggtgtgcctgattagcgatttttatccgggcgcggtgaccgtggcgtggaaagcggatagcagcccggtggcgggcgtggaaaccaccaccccgagcaaacagagcaacaacaaatatgcggcgagcagctatctgagcctgaccccggaacagtggaaaagccatcgcagctatagctgccaggtgacccatgaaggcagcaccgtggaaaaaaccgtggcgccgaccgaatgcagc

SEQ ID NO: 143 - DNA, 714 bp, synthetic construct
  misc_feature 682..714: note = /note="This region may be absent in its entirety"
  misc_feature 700..714: note = /note="This region may be absent in its entirety"
  misc_feature 1..714: note = source = /note="Description of Artificial Sequence: Synthetic polynucleotide"
  misc_feature 1..714: note = source = /note="See specification as filed for detailed description of substitutions and preferred embodiments"
  source 1..714: mol_type = other DNA
caggtgcagctggtgcagagcggcgccgaggtgaagaagcccggcgccagcgtgaaggtgagctgcaaggccagcggctacatcttcagcaactactggatccagtgggtgagacaggcccccggccagggcctggagtggatgggcgagatcctgcccggcagcggcagcaccgagtacaccgagaacttcaaggacagagtgaccatgaccagagacaccagcaccagcaccgtgtacatggagctgagcagcctgagaagcgaggacaccgccgtgtactactgcgccagatacttcttcggcagcagccccaactggtacttcgacgtgtggggccagggcaccctggtgaccgtgagcagcgccagcaccaagggccccagcgtgttccccctggccccctgcagcagaagcaccagcgagagcaccgccgccctgggctgcctggtgaaggactacttccccgagcccgtgaccgtgagctggaacagcggcgccctgaccagcggcgtgcacaccttccccgccgtgctgcagagcagcggcctgtacagcctgagcagcgtggtgaccgtgcccagcagcaacttcggcacccagacctacacctgcaacgtggaccacaagcccagcaacaccaaggtggacaagaccgtggagagaaagtgctgcgtggagtgccccccctgccccgccccccccgtggccggc

SEQ ID NO: 144 - DNA, 642 bp, synthetic construct
  misc_feature 1..642: note = source = /note="Description of Artificial Sequence: Synthetic polynucleotide"
  source 1..642: mol_type = other DNA
gacatccagatgacccagagccccagcagcctgagcgccagcgtgggcgacagagtgaccatcacctgcggcgccagcgagaacatctacggcgccctgaactggtaccagcagaagcccggcaaggcccccaagctgctgatctacggcgccaccaacctggccgacggcgtgcccagcagattcagcggcagcggcagcggcaccgacttcaccctgaccatcagcagcctgcagcccgaggacttcgccacctactactgccagaacgtgctgaacacccccctgaccttcggccagggcaccaaggtggagatcaagagaaccgtggccgcccccagcgtgttcatcttcccccccagcgacgagcagctgaagagcggcaccgccagcgtggtgtgcctgctgaacaacttctaccccagagaggccaaggtgcagtggaaggtggacaacgccctgcagagcggcaacagccaggagagcgtgaccgagcaggacagcaaggacagcacctacagcctgagcagcaccctgaccctgagcaaggccgactacgagaagcacaaggtgtacgcctgcgaggtgacccaccagggcctgagcagccccgtgaccaagagcttcaacagaggcgagtgc

SEQ ID NO: 145 - DNA, 711 bp, synthetic construct
  misc_feature 652..711: note = /note="This region may be absent in its entirety"
  misc_feature 679..711: note = /note="This region may be absent in its entirety"
  misc_feature 1..711: note = source = /note="Description of Artificial Sequence: Synthetic polynucleotide"
  misc_feature 1..711: note = source = /note="See specification as filed for detailed description of substitutions and preferred embodiments"
  source 1..711: mol_type = other DNA
caggtgcagctgcaggagagcggccccggcctggtgaagcccagcgagaccctgagcctgacctgcaccgtgagcggcttcagcctgctgagctacggcgtgcactgggtgagacagccccccggcaagggcctggagtggctgggcgtgatctggaccggcggcaccaccaactacaacagcgccctgatgagcagattcaccatcagcaaggacgacagcaagaacaccgtgtacctgaagatgaacagcctgaagaccgaggacaccgccatctactactgcgccagatactactacggcatggactactggggccagggcaccctggtgaccgtgagcagcgccagcaccaagggccccagcgtgttccccctggccccctgcagcagaagcaccagcgagagcaccgccgccctgggctgcctggtgaaggactacttccccgagcccgtgaccgtgagctggaacagcggcgccctgaccagcggcgtgcacaccttccccgccgtgctgcagagcagcggcctgtacagcctgagcagcgtggtgaccgtgcccagcagcagcctgggcaccaagacctacacctgcaacgtggaccacaagcccagcaacaccaaggtggacaagagagtggagagcaagtacggccccccctgccccccctgccccgcccccgagttcctgggcggccccagcgtgttcctg

SEQ ID NO: 146 - DNA, 642 bp, synthetic construct
  misc_feature 1..642: note = source = /note="Description of Artificial Sequence: Synthetic polynucleotide"
  source 1..642: mol_type = other DNA
gacatccagatgacccagagccccagcagcctgagcgccagcgtgggcgacagagtgaccatcacctgcaaggccagccaggacgtgagaaacaccgtggcctggtaccagcagaagcccggcaaggcccccaagctgctgatctacagcagcagctacagaaacaccggcgtgcccgacagattcagcggcagcggcagcggcaccgacttcaccctgaccatcagcagcctgcaggccgaggacgtggccgtgtactactgccagcagcactacatcaccccctacaccttcggcggcggcaccaaggtggagatcaagagaaccgtggccgcccccagcgtgttcatcttcccccccagcgacgagcagctgaagagcggcaccgccagcgtggtgtgcctgctgaacaacttctaccccagagaggccaaggtgcagtggaaggtggacaacgccctgcagagcggcaacagccaggagagcgtgaccgagcaggacagcaaggacagcacctacagcctgagcagcaccctgaccctgagcaaggccgactacgagaagcacaaggtgtacgcctgcgaggtgacccaccagggcctgagcagccccgtgaccaagagcttcaacagaggcgagtgc

SEQ ID NO: 147 - DNA, 741 bp, synthetic construct
  misc_feature 679..741: note = /note="This region may be absent in its entirety"
  variation 688..690: replace = ctg
  misc_feature 691..741: note = /note="This region may be absent in its entirety"
  misc_feature 709..741: note = /note="This region may be absent in its entirety"
  misc_feature 1..741: note = /note="Variant nucleotides given in the sequence have no preference with respect to those in the annotations for variant positions"
  misc_feature 1..741: note = source = /note="Description of Artificial Sequence: Synthetic polynucleotide"
  misc_feature 1..741: note = source = /note="See specification as filed for detailed description of substitutions and preferred embodiments"
  source 1..741: mol_type = other DNA
gaggtgcagctgctggagagcggcggcggcctggtgcagcccggcggcagcctgagactgagctgcgccgccagcggcttcaccttcagccactacatcatgatgtgggtgagacaggcccccggcaagggcctggagtgggtgagcggcatctacagcagcggcggcatcaccgtgtacgccgacagcgtgaagggcagattcaccatcagcagagacaacagcaagaacaccctgtacctgcagatgaacagcctgagagccgaggacaccgccgtgtactactgcgcctacagaagaatcggcgtgcccagaagagacgagttcgacatctggggccagggcaccatggtgaccgtgagcagcgccagcaccaagggccccagcgtgttccccctggcccccagcagcaagagcaccagcggcggcaccgccgccctgggctgcctggtgaaggactacttccccgagcccgtgaccgtgagctggaacagcggcgccctgaccagcggcgtgcacaccttccccgccgtgctgcagagcagcggcctgtacagcctgagcagcgtggtgaccgtgcccagcagcagcctgggcacccagacctacatctgcaacgtgaaccacaagcccagcaacaccaaggtggacaagagagtggagcccaagagctgcgacaagacccacacctgccccccctgccccgcccccgagctgctgggcggccccagcgtgttcctg

SEQ ID NO: 148 - DNA, 639 bp, synthetic construct
  misc_feature 1..639: note = source = /note="Description of Artificial Sequence: Synthetic polynucleotide"
  source 1..639: mol_type = other DNA
gacatccagatgacccagagccccagcaccctgagcgccagcgtgggcgacagagtgaccatcacctgcagagccagccagagcatcagcagctggctggcctggtaccagcagaagcccggcaaggcccccaagctgctgatctacaaggccagcaccctggagagcggcgtgcccagcagattcagcggcagcggcagcggcaccgagttcaccctgaccatcagcagcctgcagcccgacgacttcgccacctactactgccagcagtacaacacctactggaccttcggccagggcaccaaggtggagatcaagagaaccgtggccgcccccagcgtgttcatcttcccccccagcgacgagcagctgaagagcggcaccgccagcgtggtgtgcctgctgaacaacttctaccccagagaggccaaggtgcagtggaaggtggacaacgccctgcagagcggcaacagccaggagagcgtgaccgagcaggacagcaaggacagcacctacagcctgagcagcaccctgaccctgagcaaggccgactacgagaagcacaaggtgtacgcctgcgaggtgacccaccagggcctgagcagccccgtgaccaagagcttcaacagaggcgagtgc

SEQ ID NO: 149 - DNA, 737 bp, synthetic construct
  misc_feature 676..737: note = /note="This region may be absent in its entirety"
  variation 685..687: replace = ctg
  misc_feature 688..737: note = /note="This region may be absent in its entirety"
  misc_feature 706..737: note = /note="This region may be absent in its entirety"
  misc_feature 1..737: note = /note="Variant nucleotides given in the sequence have no preference with respect to those in the annotations for variant positions"
  misc_feature 1..737: note = source = /note="Description of Artificial Sequence: Synthetic polynucleotide"
  misc_feature 1..737: note = source = /note="See specification as filed for detailed description of substitutions and preferred embodiments"
  source 1..737: mol_type = other DNA
gaggtgcagctggtggagagcggcggcggcctggtgcagcccggcagaagcctgagactgagctgcgccgccagcggcttcaccttcgacgactacgccatgcactgggtgagacaggcccccggcaagggcctggagtgggtgagcgccatcacctggaacagcggccacatcgactacgccgacagcgtggagggcagattcaccatcagcagagacaacgccaagaacagcctgtacctgcagatgaacagcctgagagccgaggacaccgccgtgtactactgcgccaaggtgagctacctgagcaccgccagcagcctggactactggggccagggcaccctggtgaccgtgagcagcgccagcaccaagggccccagcgtgttccccctggcccccagcagcaagagcaccagcggcggcaccgccgccctgggctgcctggtgaaggactacttccccgagcccgtgaccgtgagctggaacagcggcgccctgaccagcggcgtgcacaccttccccgccgtgctgcagagcagcggcctgtacagcctgagcagcgtggtgaccgtgcccagcagcagcctgggcacccagacctacatctgcaacgtgaaccacaagcccagcaacaccaaggtggacaagaaggtggagcccaagagctgcgacaagacccacacctgccccccctgccccgccccgagctgctgggcggccccagcgtgttcctg

SEQ ID NO: 150 - DNA, 462 bp, synthetic construct
  misc_feature 1..462: note = source = /note="Description of Artificial Sequence: Synthetic polynucleotide"
  source 1..462: mol_type = other DNA
agattcagcggcagcggcagcggcaccgacttcaccctgaccatcagcagcctgcagcccgaggacgtggccacctactactgccagagatacaacagagccccctacaccttcggccagggcaccaaggtggagatcaagagaaccgtggccgcccccagcgtgttcatcttcccccccagcgacgagcagctgaagagcggcaccgccagcgtggtgtgcctgctgaacaacttctaccccagagaggccaaggtgcagtggaaggtggacaacgccctgcagagcggcaacagccaggagagcgtgaccgagcaggacagcaaggacagcacctacagcctgagcagcaccctgaccctgagcaaggccgactacgagaagcacaaggtgtacgcctgcgaggtgacccaccagggcctgagcagccccgtgaccaagagcttcaacagaggcgagtgc

SEQ ID NO: 151 - DNA, 735 bp, synthetic construct
  misc_feature 673..735: note = /note="This region may be absent in its entirety"
  variation 682..684: replace = ctg
  misc_feature 685..735: note = /note="This region may be absent in its entirety"
  misc_feature 703..735: note = /note="This region may be absent in its entirety"
  misc_feature 1..735: note = /note="Variant nucleotides given in the sequence have no preference with respect to those in the annotations for variant positions"
  misc_feature 1..735: note = source = /note="Description of Artificial Sequence: Synthetic polynucleotide"
  misc_feature 1..735: note = source = /note="See specification as filed for detailed description of substitutions and preferred embodiments"
  source 1..735: mol_type = other DNA
gaggtgaagctggaggagagcggcggcggcctggtgcagcccggcggcagcatgaagctgagctgcgtggccagcggcttcatcttcagcaaccactggatgaactgggtgagacagagccccgagaagggcctggagtgggtggccgagatcagaagcaagagcatcaacagcgccacccactacgccgagagcgtgaagggcagattcaccatcagcagagacgacagcaagagcgccgtgtacctgcagatgaccgacctgagaaccgaggacaccggcgtgtactactgcagcagaaactactacggcagcacctacgactactggggccagggcaccaccctgaccgtgagcagcgccagcaccaagggccccagcgtgttccccctggcccccagcagcaagagcaccagcggcggcaccgccgccctgggctgcctggtgaaggactacttccccgagcccgtgaccgtgagctggaacagcggcgccctgaccagcggcgtgcacaccttccccgccgtgctgcagagcagcggcctgtacagcctgagcagcgtggtgaccgtgcccagcagcagcctgggcacccagacctacatctgcaacgtgaaccacaagcccagcaacaccaaggtggacaagaaggtggagcccaagagctgcgacaagacccacacctgccccccctgccccgcccccgagctgctgggcggccccagcgtgttcctg

SEQ ID NO: 152 - DNA, 642 bp, synthetic construct
  misc_feature 1..642: note = source = /note="Description of Artificial Sequence: Synthetic polynucleotide"
  source 1..642: mol_type = other DNA
gacatcctgctgacccagagccccgccatcctgagcgtgagccccggcgagagagtgagcttcagctgcagagccagccagttcgtgggcagcagcatccactggtaccagcagagaaccaacggcagccccagactgctgatcaagtacgccagcgagagcatgagcggcatccccagcagattcagcggcagcggcagcggcaccgacttcaccctgagcatcaacaccgtggagagcgaggacatcgccgactactactgccagcagagccacagctggcccttcaccttcggcagcggcaccaacctggaggtgaagagaaccgtggccgcccccagcgtgttcatcttcccccccagcgacgagcagctgaagagcggcaccgccagcgtggtgtgcctgctgaacaacttctaccccagagaggccaaggtgcagtggaaggtggacaacgccctgcagagcggcaacagccaggagagcgtgaccgagcaggacagcaaggacagcacctacagcctgagcagcaccctgaccctgagcaaggccgactacgagaagcacaaggtgtacgcctgcgaggtgacccaccagggcctgagcagccccgtgaccaagagcttcaacagaggcgagtgc

SEQ ID NO: 153 - DNA, 711 bp, synthetic construct
  misc_feature 652..711: note = /note="This region may be absent in its entirety"
  misc_feature 679..711: note = /note="This region may be absent in its entirety"
  misc_feature 1..711: note = source = /note="Description of Artificial Sequence: Synthetic polynucleotide"
  misc_feature 1..711: note = source = /note="See specification as filed for detailed description of substitutions and preferred embodiments"
  source 1..711: mol_type = other DNA
gaggtgaaggtggtggagagcggcggcggcctggtgcagcccggcggcagcatgaagctgagctgcgtggtgagcggcttcaccttcagcaactactgggtgaactgggtgaggcaggcccccggcaagggcctggagtgggtggcccagatcaggctgaagagcgacaactacgccacccactacgaggagagcgtgaagggcaggttcaccatcagcagggacgacagcaagagcagcgtgtacctgcagatgaacaacctgagggccgaggacagcggcatctactactgcaccaactgggaggactactggggccagggcaccaccgtgaccgtgagcagcgccagcaccaagggccccagcgtgttccccctggccccctgcagcaggagcaccagcgagagcaccgccgccctgggctgcctggtgaaggactacttccccgagcccgtgaccgtgagctggaacagcggcgccctgaccagcggcgtgcacaccttccccgccgtgctgcagagcagcggcctgtacagcctgagcagcgtggtgaccgtgcccagcagcagcctgggcaccaagacctacacctgcaacgtggaccacaagcccagcaacaccaaggtggacaagagggtggagagcaagtacggccccccctgccccccctgccccgcccccgagttcctgggcggccccagcgtgttcctg

SEQ ID NO: 154 - DNA, 654 bp, synthetic construct
  misc_feature 1..654: note = source = /note="Description of Artificial Sequence: Synthetic polynucleotide"
  source 1..654: mol_type = other DNA
gacatcgtgctgacccagagccccgacagcctggccgtgagcctgggcgagagggccaccatcagctgcagggccagccagagcgtgagcaccagcaggtacagctacatccactggtaccagcagaagcccggccagccccccaagctgctgatcaagtacgccagcaacctggagagcggcgtgcccagcaggttcagcggcagcggcagcggcaccgacttcaccctgaacatccaccccctggagcccgaggacttcgccacctactactgccaccacagctgggagatccccctgaccttcggccagggcaccaagctggagatcaagaggaccgtggccgcccccagcgtgttcatcttcccccccagcgacgagcagctgaagagcggcaccgccagcgtggtgtgcctgctgaacaacttctaccccagggaggccaaggtgcagtggaaggtggacaacgccctgcagagcggcaacagccaggagagcgtgaccgagcaggacagcaaggacagcacctacagcctgagcagcaccctgaccctgagcaaggccgactacgagaagcacaaggtgtacgcctgcgaggtgacccaccagggcctgagcagccccgtgaccaagagcttcaacaggggcgagtgc

SEQ ID NO: 155 - DNA, 738 bp, synthetic construct
  misc_feature 1..738: note = source = /note="Description of Artificial Sequence: Synthetic polynucleotide"
  source 1..738: mol_type = other DNA
caggtgcagctggtggagagcggcggcggcgtggtgcagcccggcagaagcctgagactgagctgcgccgccagcggcttcaccttcagcagcttcggcatgcactgggtgagacaggcccccggcaagggcctggagtgggtggccgtgatcagcttcgacggcagcatcaagtacagcgtggacagcgtgaagggcagattcaccatcagcagagacaacagcaagaacaccctgttcctgcagatgaacagcctgagagccgaggacaccgccgtgtactactgcgccagagacagactgaactactacgacagcagcggctactaccactacaagtactacggcatggccgtgtggggccagggcaccaccgtgaccgtgagcagcgccagcaccaagggccccagcgtgttccccctggccccctgcagcagaagcaccagcgagagcaccgccgccctgggctgcctggtgaaggactacttccccgagcccgtgaccgtgagctggaacagcggcgccctgaccagcggcgtgcacaccttccccgccgtgctgcagagcagcggcctgtacagcctgagcagcgtggtgaccgtgcccagcagcaacttcggcacccagacctacacctgcaacgtggaccacaagcccagcaacaccaaggtggacaagaccgtggagagaaagtgctgcgtggagtgccccccctgccccgccccccccgtggccggc

SEQ ID NO: 156 - DNA, 648 bp, synthetic construct
  misc_feature 1..648: note = source = /note="Description of Artificial Sequence: Synthetic polynucleotide"
  source 1..648: mol_type = other DNA
cagagcgtgctgacccagccccccagcgtgagcgccgcccccggccagaaggtgaccatcagctgcagcggcagcagcagcaacatcggcaacaactacgtgagctggtaccagcagctgcccggcaccgcccccaagctgctgatctacgacaacaacaagagacccagcggcatccccgacagattcagcggcagcaagagcggcaccagcaccaccctgggcatcaccggcctgcagaccggcgacgaggccgactactactgcggcacctgggacagcagactgagcgccgtggtgttcggcggcggcaccaagctgaccgtgctgggccagcccaaggccaaccccaccgtgaccctgttcccccccagcagcgaggagctgcaggccaacaaggccaccctggtgtgcctgatcagcgacttctaccccggcgccgtgaccgtggcctggaaggccgacggcagccccgtgaaggccggcgtggagaccaccaagcccagcaagcagagcaacaacaagtacgccgccagcagctacctgagcctgacccccgagcagtggaagagccacagaagctacagctgccaggtgacccacgagggcagcaccgtggagaagaccgtggcccccaccgagtgcagc

SEQ ID NO: 157 - DNA, 731 bp, synthetic construct
  misc_feature 685..731: note = /note="This region may be absent in its entirety"
  variation 694..696: replace = ctg
  misc_feature 697..731: note = /note="This region may be absent in its entirety"
  misc_feature 715..731: note = /note="This region may be absent in its entirety"
  misc_feature 1..731: note = /note="Variant nucleotides given in the sequence have no preference with respect to those in the annotations for variant positions"
  misc_feature 1..731: note = source = /note="Description of Artificial Sequence: Synthetic polynucleotide"
  misc_feature 1..731: note = source = /note="See specification as filed for detailed description of substitutions and preferred embodiments"
  source 1..731: mol_type = other DNA
gaggtgcagctggtggagagcggcggcggcctggtgcagcccggcggcagcctgaggctgagctgcagcgccagcggcttcaccttcagcagcttcggcatgcactgggtgaggcaggcccccggcaagggcctggagtgggtggcctacatcagcagcggcagcagcaccatctactacggcgacaccgtgaagggcaggttcaccatcagcagggacaacgccaagaacagcctgttcctgcagatgagcagcctgagggccgaggacaccgccgtgtactactgcgccagggagggcggctactactacggcaggagctactacaccatggactactggggccagggcaccaccgtgaccgtgagcagcgccagcaccaagggccccagcgtgttccccctggcccccagcagcaagagcaccagcggcggcaccgccgccctgggctgcctggtgaaggactacttccccgagcccgtgaccgtgagctggaacagcggcgccctgaccagcggcgtgcacaccttccccgccgtgctgcagagcagcggcctgtacagcctgagcagcgtggtgaccgtgcccagcagcagcctgggcacccagacctacatctgcaacgtgaaccacaagcccagcaacaccaaggtggacaagaaggtggagcccaagagctgcgacaagacccacacctgccccccctgccccgccccgagctgctgggcggc

SEQ ID NO: 158 - DNA, 657 bp, synthetic construct
  misc_feature 1..657: note = source = /note="Description of Artificial Sequence: Synthetic polynucleotide"
  source 1..657: mol_type = other DNA
gacgtggtgatgacccagagccccctgagcctgcccgtgacccccggcgcccccgccagcatcagctgcaggagcagccagagcatcgtgcacagcaacggcaacacctacctggagtggtacctgcagaagcccggccagagccccaagctgctgatctacaaggtgagcaacaggttcagcggcgtgcccgacaggttcagcggcagcggcagcggcaccgacttcaccctgaggatcagcagggtggaggccgaggacgtgggcatctactactgcttccagggcagccacgtgccccccaccttcggccccggcaccaagctggagatcaagaggaccgtggccgcccccagcgtgttcatcttcccccccagcgacgagcagctgaagagcggcaccgccagcgtggtgtgcctgctgaacaacttctaccccagggaggccaaggtgcagtggaaggtggacaacgccctgcagagcggcaacagccaggagagcgtgaccgagcaggacagcaaggacagcacctacagcctgagcagcaccctgaccctgagcaaggccgactacgagaagcacaaggtgtacgcctgcgaggtgacccaccagggcctgagcagccccgtgaccaagagcttcaacaggggcgagtgc

SEQ ID NO: 159 - DNA, 369 bp, synthetic construct
  misc_feature 1..369: note = source = /note="Description of Artificial Sequence: Synthetic polynucleotide"
  source 1..369: mol_type = other DNA
gaggtgaagctggtggagagcggcggcggcctggtgcagcccggcggcagcctgaggctgagctgcgccaccagcggcttcaccttcagcgacttctacatggagtgggtgaggcaggcccccggcaagaggctggagtggatcgccgccagcaggaacaaggccaacgactacaccaccgagtacgccgacagcgtgaagggcaggttcatcgtgagcagggacaccagccagagcatcctgtacctgcagatgaacgccctgagggccgaggacaccgccatctactactgcgccagggactactacggcagcagctactggtacttcgacgtgtggggcgccggcaccaccgtgaccgtgagcagc

SEQ ID NO: 160 - DNA, 339 bp, synthetic construct
  misc_feature 1..339: note = source = /note="Description of Artificial Sequence: Synthetic polynucleotide"
  source 1..339: mol_type = other DNA
gacatcgtgatgacccagagccccagcagcctgagcgtgagcgccggcaagaaggtgaccatcagctgcaccgccagcgagagcctgtacagcagcaagcacaaggtgcactacctggcctggtaccagaagaagcccgagcagagccccaagctgctgatctacggcgccagcaacaggtacatcggcgtgcccgacaggttcaccggcagcggcagcggcaccgacttcaccctgaccatcagcagcgtgcaggtggaggacctgacccactactactgcgcccagttctacagctaccccctgaccttcggcgccggcaccaagctggagatcaag

SEQ ID NO: 161 - protein, 20 aa, unidentified
  REGION 1..20: note = source = /note="Description of Unknown: signal sequence"
MYRMQLLLLIALSLALVTNS

SEQ ID NO: 162 - protein, 7 aa, synthetic construct
  REGION 1..7: note = source = /note="Description of Artificial Sequence: Synthetic peptide"
LGETTRP

SEQ ID NO: 163 - protein, 9 aa, synthetic construct
  REGION 1..9: note = source = /note="Description of Artificial Sequence: Synthetic peptide"
LALGETTRP

SEQ ID NO: 164 - protein, 26 aa, unidentified
  REGION 1..26: note = source = /note="Description of Unknown: VEGF-A signal peptide"
MNFLLSWVHWSLALLLYLHHAKWSQA

SEQ ID NO: 165 - protein, 29 aa, unidentified
  REGION 1..29: note = source = /note="Description of Unknown: Fibulin-1 signal peptide"
MERAAPSRRVPLPLLLLGGLALLAAGVDA

SEQ ID NO: 166 - protein, 19 aa, unidentified
  REGION 1..19: note = source = /note="Description of Unknown: Vitronectin signal peptide"
MAPLRPLLILALLAWVALA

SEQ ID NO: 167 - protein, 18 aa, unidentified
  REGION 1..18: note = source = /note="Description of Unknown: Complement Factor H signal peptide"
MRLLAKIICLMLWAICVA

SEQ ID NO: 168 - protein, 19 aa, unidentified
  REGION 1..19: note = source = /note="Description of Unknown: Opticin signal peptide"
MRLLAFLSLLALVLQETGT

SEQ ID NO: 169 - protein, 18 aa, unidentified
  REGION 1..18: note = source = /note="Description of Unknown: Albumin signal peptide"
MKWVTFISLLFLFSSAYS

SEQ ID NO: 170 - protein, 18 aa, unidentified
  REGION 1..18: note = source = /note="Description of Unknown: Chymotrypsinogen signal peptide"
MAFLWLLSCWALLGTTFG

SEQ ID NO: 171 - protein, 20 aa, unidentified
  REGION 1..20: note = source = /note="Description of Unknown: Interleukin-2 signal peptide"
MYRMQLLSCIALILALVTNS

SEQ ID NO: 172 - protein, 15 aa, unidentified
  REGION 1..15: note = source = /note="Description of Unknown: Trypsinogen-2 signal peptide"
MNLLLILTFVAAAVA

SEQ ID NO: 173 - protein, 17 aa, Homo sapiens
MRAWIFFLLCLAGRALA

SEQ ID NO: 174 - protein, 22 aa, Homo sapiens
MFSFVDLRLLLLLAATALLTHG

SEQ ID NO: 175 - protein, 19 aa, Homo sapiens
MKLVFLVLLFLGALGLCLA

SEQ ID NO: 176 - protein, 22 aa, Homo sapiens
MGPTSGPSLLLLLLTHLPLALG

SEQ ID NO: 177 - protein, 18 aa, Homo sapiens
MSLSAFTLFLALIGGTSG

SEQ ID NO: 178 - protein, 27 aa, Homo sapiens
MAPHRPAPALLCALSLALCALSLPVRA

SEQ ID NO: 179 - protein, 22 aa, Homo sapiens
MWATLPLLCAGAWLLGVPVCGA

SEQ ID NO: 180 - protein, 19 aa, Homo sapiens
MQALVLLLCIGALLGHSSC

SEQ ID NO: 181 - protein, 23 aa, Homo sapiens
MQMSPALTCLVLGLALVFGEGSA

SEQ ID NO: 182 - protein, 20 aa, Homo sapiens
MQPSSLLPLALCLLAAPASA

SEQ ID NO: 183 - protein, 23 aa, Homo sapiens
MAPFEPLASGILLLLWLIAPSRA

SEQ ID NO: 184 - protein, 31 aa, Homo sapiens
MLRGPGPGLLLLAVQCLGTAVPSTGASKSKR

SEQ ID NO: 185 - protein, 15 aa, Homo sapiens
MWCIVLFSLLAWVYA

SEQ ID NO: 186 - protein, 17 aa, Homo sapiens
MNPTLILAAFCLGIASA

SEQ ID NO: 187 - protein, 17 aa, Homo sapiens
MWQLWASLCCLLVLANA

SEQ ID NO: 188 - protein, 16 aa, Homo sapiens
MLLILLSVALLAFSSA

SEQ ID NO: 189 - protein, 20 aa, Homo sapiens
MWKRWLALALALVAVAWVRA

SEQ ID NO: 190 - protein, 24 aa, Homo sapiens
MPSSVSWGILLLAGLCCLVPVSLA

SEQ ID NO: 191 - protein, 18 aa, Homo sapiens
MKAAVLTLAVLFLTGSQA

SEQ ID NO: 192 - protein, 18 aa, Homo sapiens
MKLLAATVLLLTICSLEG

SEQ ID NO: 193 - protein, 27 aa, Homo sapiens
MDPPRPALLALLALPALLLLLLAGARA

SEQ ID NO: 194 - protein, 28 aa, Homo sapiens
MQRVNMIMAESPGLITICLLGYLLSAEC

SEQ ID NO: 195 - protein, 20 aa, Homo sapiens
MGPLMVLFCLLFLYPGLADS

SEQ ID NO: 196 - protein, 18 aa, Homo sapiens
MWLLVSVILISRISSVGG

SEQ ID NO: 197 - protein, 18 aa, Homo sapiens
MLLLFSVILISWVSTVGG

SEQ ID NO: 198 - protein, 19 aa, Homo sapiens
MFSMRIVCLVLSVVGTAWT

SEQ ID NO: 199 - protein, 30 aa, Homo sapiens
MKRMVSWSFHKLKTMKHLLLLLLCVFLVKS

SEQ ID NO: 200 - protein, 26 aa, Homo sapiens
MSWSLHPRNLILYFYALLFLSSTCVA

SEQ ID NO: 201 - protein, 18 aa, Homo sapiens
MKSLVLLLCLAQLWGCHS

SEQ ID NO: 202 - protein, 23 aa, Homo sapiens
MARVLGAPVALGLWSLCWSLAIA

SEQ ID NO: 203 - protein, 18 aa, Homo sapiens
MKLITILFLCSRLLLSLT

SEQ ID NO: 204 - protein, 20 aa, Homo sapiens
MSLFPSLPLLLLSMVAASYS

SEQ ID NO: 205 - protein, 19 aa, Homo sapiens
MEHKEVVLLLLLFLKSGQG

SEQ ID NO: 206 - protein, 24 aa, Homo sapiens
MAHVRGLQLPGCLALAALCSLVHS

SEQ ID NO: 207 - protein, 29 aa, Homo sapiens
MISRMEKMTMMMKILIMFALGMNYWSCSG

SEQ ID NO: 208 - protein, 32 aa, Homo sapiens
MYSNVIGTVTSGKRKVYLLSLLLIGFWDCVTC

SEQ ID NO: 209 - protein, 19 aa, Homo sapiens
MRLAVGALLVCAVLGLCLA

SEQ ID NO: 210 - protein, 19 aa, synthetic construct
  REGION 1..19: note = source = /note="Description of Artificial Sequence: Synthetic peptide"
LLNFDLLKLAGDVESNPGP

SEQ ID NO: 211 - protein, 21 aa, synthetic construct
  VARIANT 1..3: note = /replace=" "
  SITE 1..21: note = /note="Variant residues given in the sequence have no preference with respect to those in the annotations for variant positions"
  REGION 1..21: note = source = /note="Description of Artificial Sequence: Synthetic peptide"
GSGEGRGSLLTCGDVEENPGP

SEQ ID NO: 212 - protein, 22 aa, synthetic construct
  VARIANT 1..3: note = /replace=" "
  SITE 1..22: note = /note="Variant residues given in the sequence have no preference with respect to those in the annotations for variant positions"
  REGION 1..22: note = source = /note="Description of Artificial Sequence: Synthetic peptide"
GSGATNFSLLKQAGDVEENPGP

SEQ ID NO: 213 - protein, 23 aa, synthetic construct
  VARIANT 1..3: note = /replace=" "
  SITE 1..23: note = /note="Variant residues given in the sequence have no preference with respect to those in the annotations for variant positions"
  REGION 1..23: note = source = /note="Description of Artificial Sequence: Synthetic peptide"
GSGQCTNYALLKLAGDVESNPGP

SEQ ID NO: 214 - protein, 25 aa, synthetic construct
  VARIANT 1..3: note = /replace=" "
  SITE 1..25: note = /note="Variant residues given in the sequence have no preference with respect to those in the annotations for variant positions"
  REGION 1..25: note = source = /note="Description of Artificial Sequence: Synthetic peptide"
GSGVKQTLNFDLLKLAGDVESNPGP

SEQ ID NO: 215 - protein, 4 aa, synthetic construct
  REGION 1..4: note = source = /note="Description of Artificial Sequence: Synthetic peptide"
RKRR

SEQ ID NO: 216 - protein, 4 aa, synthetic construct
  REGION 1..4: note = source = /note="Description of Artificial Sequence: Synthetic peptide"
RRRR

SEQ ID NO: 217 - protein, 4 aa, synthetic construct
  REGION 1..4: note = source = /note="Description of Artificial Sequence: Synthetic peptide"
RRKR

SEQ ID NO: 218 - protein, 4 aa, synthetic construct
  REGION 1..4: note = source = /note="Description of Artificial Sequence: Synthetic peptide"
RKKR

SEQ ID NO: 219 - protein, 6 aa, synthetic construct
  REGION 1..6: note = source = /note="Description of Artificial Sequence: Synthetic peptide"
CPPCPA

SEQ ID NO: 220 - protein, 5 aa, synthetic construct
  REGION 1..5: note = source = /note="Description of Artificial Sequence: Synthetic peptide"
CPPCP

SEQ ID NO: 221 - protein, 5 aa, synthetic construct
  REGION 1..5: note = source = /note="Description of Artificial Sequence: Synthetic peptide"
CPPCA

SEQ ID NO: 222 - protein, 16 aa, synthetic construct
  REGION 1..16: note = source = /note="Description of Artificial Sequence: Synthetic peptide"
KTHTCPPCPAPELLGG

SEQ ID NO: 223 - protein, 4 aa, synthetic construct
  REGION 1..4: note = source = /note="Description of Artificial Sequence: Synthetic peptide"
KTHL

SEQ ID NO: 224 - protein, 4 aa, synthetic construct
  REGION 1..4: note = source = /note="Description of Artificial Sequence: Synthetic peptide"
KTHT

SEQ ID NO: 225 - protein, 10 aa, synthetic construct
  REGION 1..10: note = source = /note="Description of Artificial Sequence: Synthetic peptide"
KTHTCPPCPA

SEQ ID NO: 226 - protein, 10 aa, synthetic construct
  REGION 1..10: note = source = /note="Description of Artificial Sequence: Synthetic peptide"
KTHLCPPCPA

SEQ ID NO: 227 - protein, 21 aa, synthetic construct
  REGION 1..21: note = source = /note="Description of Artificial Sequence: Synthetic peptide"
KTHTCPPCPAPELLGGPSVFL

SEQ ID NO: 228 - protein, 21 aa, synthetic construct
  REGION 1..21: note = source = /note="Description of Artificial Sequence: Synthetic peptide"
KTHLCPPCPAPELLGGPSVFL

SEQ ID NO: 229 - protein, 9 aa, synthetic construct
  REGION 1..9: note = source = /note="Description of Artificial Sequence: Synthetic peptide"
GPPCPPCPA

SEQ ID NO: 230 - protein, 20 aa, synthetic construct
  REGION 1..20: note = source = /note="Description of Artificial Sequence: Synthetic peptide"
GPPCPPCPAPEFLGGPSVFL

SEQ ID NO: 231 - protein, 15 aa, synthetic construct
  REGION 1..15: note = source = /note="Description of Artificial Sequence: Synthetic peptide"
GPPCPPCPAPEFLGG

SEQ ID NO: 232 - protein, 12 aa, synthetic construct
  REGION 1..12: note = source = /note="Description of Artificial Sequence: Synthetic peptide"
CPPCPAPPVAGG

SEQ ID NO: 233 - protein, 11 aa, synthetic construct
  REGION 1..11: note = source = /note="Description of Artificial Sequence: Synthetic peptide"
CPPCPAPPVAG

SEQ ID NO: 234 - protein, 213 aa, synthetic construct
  REGION 1..213: note = source = /note="Description of Artificial Sequence: Synthetic polypeptide"
IQMTQSPSSLSASVGDRVTITCKASQDVRNTVAWYQQKPGKAPKLLIYSSSYRNTGVPDRFSGSGSGTDFTLTISSLQAEDVAVYYCQQHYITPYTFGGGTKVEIKRTVAAPSVFIFPPSDEQLKSGTASVVCLLNNFYPREAKVQWKVDNALQSGNSQESVTEQDSKDSTYSLSSTLTLSKADYEKHKVYACEVTHQGLSSPVTKSFNRGEC

SEQ ID NO: 235 - protein, 213 aa, synthetic construct
  REGION 1..213: note = source = /note="Description of Artificial Sequence: Synthetic polypeptide"
DILLTQSPAILSVSPGERVSFSCRASQFVSSIHWYQQRTNGSPRLLIKYASESMSGIPSRFSGSGSGTDFTLSINTVESEDIADYYCQQSHSWPFTFGSGTNLEVKRTVAAPSVFIFPPSDEQLKSGTASVVCLLNNFYPREAKVQWKVDNALQSGNSQESVTEQDSKDSTYSLSSTLTLSKADYEKHKVYACEVTHQGLSSPVTKSFNRGEC

SEQ ID NO: 236 - protein, 16 aa, synthetic construct
  REGION 1..16: note = source = /note="Description of Artificial Sequence: Synthetic peptide"
KTHTCPPCPAPELAGA

SEQ ID NO: 237 - protein, 21 aa, synthetic construct
  REGION 1..21: note = source = /note="Description of Artificial Sequence: Synthetic peptide"
KTHTCPPCPAPELAGAPSVFL

SEQ ID NO: 238 - protein, 21 aa, synthetic construct
  REGION 1..21: note = source = /note="Description of Artificial Sequence: Synthetic peptide"
KTHLCPPCPAPELAGAPSVFL

SEQ ID NO: 239 - protein, 16 aa, synthetic construct
  REGION 1..16: note = source = /note="Description of Artificial Sequence: Synthetic peptide"
KTHLCPPCPAPELLGG

SEQ ID NO: 240 - protein, 14 aa, synthetic construct
  REGION 1..14: note = source = /note="Description of Artificial Sequence: Synthetic peptide"
GPPCPPCPAPEFLG

SEQ ID NO: 241 - protein, 19 aa, synthetic construct
  REGION 1..19: note = source = /note="Description of Artificial Sequence: Synthetic peptide"
GPPCPPCPAPEFLGPSVFL

SEQ ID NO: 242 - protein, 28 aa, synthetic construct
  REGION 1..28: note = source = /note="Description of Artificial Sequence: Synthetic peptide"
RKRRAPVKQTLNFDLLKLAGDVESNPGP

SEQ ID NO: 243 - protein, 30 aa, synthetic construct
  SITE 1..30: note = /note="This sequence may encompass 1-6 'Gly Gly Gly Gly Ser' repeating units"
  REGION 1..30: note = source = /note="Description of Artificial Sequence: Synthetic polypeptide"
GGGGSGGGGSGGGGSGGGGSGGGGSGGGGS

SEQ ID NO: 244 - protein, 19 aa, unidentified
  REGION 1..19: note = source = /note="Description of Unknown: signal sequence"
MYRMQLLLIALSLALVTNS

SEQ ID NO: 245 - protein, 15 aa, synthetic construct
  REGION 1..15: note = source = /note="Description of Artificial Sequence: Synthetic peptide"
GGGGSGGGGSGGGGS

SEQ ID NO: 246 - protein, 20 aa, synthetic construct
  REGION 1..20: note = source = /note="Description of Artificial Sequence: Synthetic peptide"
GGGGSGGGGSGGGGSGGGGS

SEQ ID NO: 247 - protein, 214 aa, synthetic construct
  REGION 1..214: note = source = /note="Description of Artificial Sequence: Synthetic polypeptide"
DIQMTQSPSSLSASVGDRVTITCRASQGIRNYLAWYQQKPGKAPKLLIYAASTLQSGVPSRFSGSGSGTDFTLTISSLQPEDVATYYCQRYNRAPYTFGQGTKVEIKRTVAAPSVFIFPPSDEQLKSGTASVVCLLNNFYPREAKVQWKVDNALQSGNSQESVTEQDSKDSTYSLSSTLTLSKADYEKHKVYACEVTHQGLSSPVTKSFNRGEC

SEQ ID NO: 248 - protein, 7 aa, synthetic construct
  REGION 1..7: note = source = /note="Description of Artificial Sequence: Synthetic peptide"
EDTAVYY

SEQ ID NO: 249 - protein, 17 aa, synthetic construct
  REGION 1..17: note = source = /note="Description of Artificial Sequence: Synthetic peptide"
DKTHTCPPCPAPELLGG

SEQ ID NO: 250 - protein, 7 aa, synthetic construct
  REGION 1..7: note = source = /note="Description of Artificial Sequence: Synthetic peptide"
EDFATYY

SEQ ID NO: 251 - protein, 7 aa, synthetic construct
  REGION 1..7: note = source = /note="Description of Artificial Sequence: Synthetic peptide"
EDVGVYY

SEQ ID NO: 252 - protein, 6 aa, synthetic construct
  REGION 1..6: note = source = /note="Description of Artificial Sequence: Synthetic peptide"
NWEDYW

SEQ ID NO: 253 - protein, 13 aa, synthetic construct
  REGION 1..13: note = source = /note="Description of Artificial Sequence: Synthetic peptide"
VECPPCPAPPVAG

SEQ ID NO: 254 - protein, 17 aa, synthetic construct
  REGION 1..17: note = source = /note="Description of Artificial Sequence: Synthetic peptide"
DKTHLCPPCPAPELLGG

SEQ ID NO: 255 - protein, 6 aa, synthetic construct
  REGION 1..6: note = source = /note="Description of Artificial Sequence: Synthetic peptide"
EDVGIY

SEQ ID NO: 256 - protein, 7 aa, synthetic construct
  REGION 1..7: note = source = /note="Description of Artificial Sequence: Synthetic peptide"
GDEADYY

SEQ ID NO: 257 - protein, 7 aa, synthetic construct
  REGION 1..7: note = source = /note="Description of Artificial Sequence: Synthetic peptide"
EDVGFYY

SEQ ID NO: 258 - protein, 10 aa, synthetic construct
  REGION 1..10: note = source = /note="Description of Artificial Sequence: Synthetic peptide"
DILTDYYIHY

SEQ ID NO: 259 - protein, 7 aa, synthetic construct
  REGION 1..7: note = source = /note="Description of Artificial Sequence: Synthetic peptide"
EDFAVYY

SEQ ID NO: 260 - protein, 6 aa, synthetic construct
  REGION 1..6: note = source = /note="Description of Artificial Sequence: Synthetic peptide"
DTATYY

SEQ ID NO: 261 - protein, 7 aa, synthetic construct
  REGION 1..7: note = source = /note="Description of Artificial Sequence: Synthetic peptide"
EDVAVYY

SEQ ID NO: 262 - protein, 9 aa, synthetic construct
  REGION 1..9: note = source = /note="Description of Artificial Sequence: Synthetic peptide"
DGWDYAIDY

SEQ ID NO: 263 - protein, 17 aa, synthetic construct
  REGION 1..17: note = source = /note="Description of Artificial Sequence: Synthetic peptide"
DKTHTCPPCPAPELAGA

SEQ ID NO: 264 - protein, 7 aa, synthetic construct
  REGION 1..7: note = source = /note="Description of Artificial Sequence: Synthetic peptide"
EDIATYY

SEQ ID NO: 265 - protein, 7 aa, synthetic construct
  REGION 1..7: note = source = /note="Description of Artificial Sequence: Synthetic peptide"
DDTAVYY

SEQ ID NO: 266 - protein, 7 aa, synthetic construct
  REGION 1..7: note = source = /note="Description of Artificial Sequence: Synthetic peptide"
EDEADYY

SEQ ID NO: 267 - protein, 7 aa, synthetic construct
  REGION 1..7: note = source = /note="Description of Artificial Sequence: Synthetic peptide"
EDTAFFY

SEQ ID NO: 268 - protein, 12 aa, synthetic construct
  REGION 1..12: note = source = /note="Description of Artificial Sequence: Synthetic peptide"
CPPCPAPEFLGG

SEQ ID NO: 269 - protein, 7 aa, synthetic construct
  REGION 1..7: note = source = /note="Description of Artificial Sequence: Synthetic peptide"
DDFATYY

SEQ ID NO: 270 - protein, 6 aa, synthetic construct
  REGION 1..6: note = source = /note="Description of Artificial Sequence: Synthetic peptide"
YQKKPE

SEQ ID NO: 271 - protein, 6 aa, synthetic construct
  REGION 1..6: note = source = /note="Description of Artificial Sequence: Synthetic peptide"
DYTTEY

SEQ ID NO: 272 - protein, 7 aa, synthetic construct
  REGION 1..7: note = source = /note="Description of Artificial Sequence: Synthetic peptide"
EDTAIYY

SEQ ID NO: 273 - protein, 7 aa, synthetic construct
  REGION 1..7: note = source = /note="Description of Artificial Sequence: Synthetic peptide"
EDFAVFY

SEQ ID NO: 274 - protein, 7 aa, synthetic construct
  REGION 1..7: note = source = /note="Description of Artificial Sequence: Synthetic peptide"
EDVATYY

SEQ ID NO: 275 - protein, 6 aa, synthetic construct
  REGION 1..6: note = source = /note="Description of Artificial Sequence: Synthetic peptide"
TFGQGT

SEQ ID NO: 276 - protein, 8 aa, synthetic construct
  REGION 1..8: note = source = /note="Description of Artificial Sequence: Synthetic peptide"
ETTYADDF

SEQ ID NO: 277 - protein, 7 aa, synthetic construct
  REGION 1..7: note = source = /note="Description of Artificial Sequence: Synthetic peptide"
SKTDYYY

SEQ ID NO: 278 - protein, 6 aa, synthetic construct
  REGION 1..6: note = source = /note="Description of Artificial Sequence: Synthetic peptide"
DDDPYY

SEQ ID NO: 279 - protein, 7 aa, synthetic construct
  REGION 1..7: note = source = /note="Description of Artificial Sequence: Synthetic peptide"
DDTAIYY

SEQ ID NO: 280 - protein, 7 aa, synthetic construct
  REGION 1..7: note = source = /note="Description of Artificial Sequence: Synthetic peptide"
FTFDDYA

SEQ ID NO: 281 - protein, 7 aa, synthetic construct
  REGION 1..7: note = source = /note="Description of Artificial Sequence: Synthetic peptide"
EDTGVYY

SEQ ID NO: 282 - protein, 7 aa, synthetic construct
  REGION 1..7: note = source = /note="Description of Artificial Sequence: Synthetic peptide"
EDIADYY

SEQ ID NO: 283 - protein, 232 aa, synthetic construct
  MOD_RES 1: note = Any amino acid
  REGION 1..232: note = source = /note="Description of Artificial Sequence: Synthetic polypeptide"
XVQLVESGGGVVQPGRSLRLSCAASGFAFSSYGMHWVRQAPGKGLEWVAVIWFDGTKKYYTDSVKGRFTISRDNSKNTLYLQMNTLRAEDTAVYYCARDRGIGARRGPYYMDVWGKGTTVTVSSASTKGPSVFPLAPSSKSTSGGTAALGCLVKDYFPEPVTVSWNSGALTSGVHTFPAVLQSSGLYSLSSVVTVPSSSLGTQTYICNVNHKPSNTKVDKRVEPKSCDKTHT

SEQ ID NO: 284 - protein, 217 aa, synthetic construct
  REGION 1..217: note = source = /note="Description of Artificial Sequence: Synthetic polypeptide"
EVQLVESGGGLVQPGGSLRLSCAASGFTFSSYGMSWVRQAPGKGLELVASINSNGGSTYYPDSVKGRFTISRDNAKNSLYLQMNSLRAEDTAVYYCASGDYWGQGTTVTVSSASTKGPSVFPLAPCSRSTSESTAALGCLVKDYFPEPVTVSWNSGALTSGVHTFPAVLQSSGLYSLSSVVTVPSSSLGTKTYTCNVDHKPSNTKVDKRVESKYGPP

SEQ ID NO: 285 - protein, 234 aa, synthetic construct
  REGION 1..234: note = source = /note="Description of Artificial Sequence: Synthetic polypeptide"
QVELVESGGGLVQPGGSLRLSCAASGFTFSSYAMSWVRQAPGKGLEWVSAINASGTRTYYADSVKGRFTISRDNSKNTLYLQMNSLRAEDTAVYYCARGKGNTHKPYGYVRYFDVWGQGTLVTVSSASTKGPSVFPLAPSSKSTSGGTAALGCLVKDYFPEPVTVSWNSGALTSGVHTFPAVLQSSGLYSLSSVVTVPSSSLGTQTYICNVNHKPSNTKVDKKVEPKSCDKTHT

SEQ ID NO: 286 - protein, 230 aa, synthetic construct
  REGION 1..230: note = source = /note="Description of Artificial Sequence: Synthetic polypeptide"
EVQLVESGGGLEQPGGSLRLSCAGSGFTFRDYAMTWVRQAPGKGLEWVSSISGSGGNTYYADSVKGRFTISRDNSKNTLYLQMNSLRAEDTAVYYCAKDRLSITIRPRYYGLDVWGQGTTVTVSSASTKGPSVFPLAPCSRSTSESTAALGCLVKDYFPEPVTVSWNSGALTSGVHTFPAVLQSSGLYSLSSVVTVPSSSLGTKTYTCNVDHKPSNTKVDKRVESKYGPP

SEQ ID NO: 287 - protein, 224 aa, synthetic construct
  REGION 1..224: note = source = /note="Description of Artificial Sequence: Synthetic polypeptide"
QVQLVQSGAEVKKPGSSVKVSCKASGYSFTDYHIHWVRQAPGQGLEWMGVINPMYGTTDYNQRFKGRVTITADESTSTAYMELSSLRSEDTAVYYCARYDYFTGTGVYWGQGTLVTVSSASTKGPSVFPLAPCSRSTSESTAALGCLVKDYFPEPVTVSWNSGALTSGVHTFPAVLQSSGLYSLSSVVTVPSSSLGTKTYTCNVDHKPSNTKVDKRVESKYGPP

SEQ ID NO: 288 - protein, 235 aa, synthetic construct
  REGION 1..235: note = source = /note="Description of Artificial Sequence: Synthetic polypeptide"
EVQLVESGGGLVQPGGSLRLSCAASGFTFSNYWMNWVRQAPGKGLEWVAAINQDGSEKYYVGSVKGRFTISRDNAKNSLYLQMNSLRVEDTAVYYCVRDYYDILTDYYIHYWYFDLWGRGTLVTVSSASTKGPSVFPLAPSSKSTSGGTAALGCLVKDYFPEPVTVSWNSGALTSGVHTFPAVLQSSGLYSLSSVVTVPSSSLGTQTYICNVNHKPSNTKVDKRVEPKSCDKTHT

SEQ ID NO: 289 - protein, 227 aa, synthetic construct
  REGION 1..227: note = source = /note="Description of Artificial Sequence: Synthetic polypeptide"
EVQLVQSGAEVKKPGESLKISCKGSGYSFTTYWLGWVRQMPGKGLDWIGIMSPVDSDIRYSPSFQGQVTMSVDKSITTAYLQWNSLKASDTAMYYCARRRPGQGYFDFWGQGTLVTVSSSSTKGPSVFPLAPSSKSTSGGTAALGCLVKDYFPEPVTVSWNSGALTSGVHTFPAVLQSSGLYSLSSVVTVPSSSLGTQTYICNVNHKPSNTKVDKRVEPKSCDKTHT

SEQ ID NO: 290 - protein, 227 aa, synthetic construct
  REGION 1..227: note = source = /note="Description of Artificial Sequence: Synthetic polypeptide"
QVTLRESGPALVKPTQTLTLTCTVSGFSLTSYSVHWVRQPPGKGLEWLGVIWASGGTDYNSALMSRLSISKDTSRNQVVLTMTNMDPVDTATYYCARDPPSSLLRLDYWGRGTPVTVSSASTKGPSVFPLAPSSKSTSGGTAALGCLVKDYFPEPVTVSWNSGALTSGVHTFPAVLQSSGLYSLSSVVTVPSSSLGTQTYICNVNHKPSNTKVDKRVEPKSCDKTHT

SEQ ID NO: 291 - protein, 229 aa, synthetic construct
  REGION 1..229: note = source = /note="Description of Artificial Sequence: Synthetic polypeptide"
QVQLVQSGAEVKKPGASVKVSCKGSGYTFTSYWMHWVRQAPGQRLEWIGEIDPSESNTNYNQKFKGRVTLTVDISASTAYMELSSLRSEDTAVYYCARGGYDGWDYAIDYWGQGTLVTVSSASTKGPSVFPLAPSSKSTSGGTAALGCLVKDYFPEPVTVSWNSGALTSGVHTFPAVLQSSGLYSLSSVVTVPSSSLGTQTYICNVNHKPSNTKVDKKVEPKSCDKTHT

SEQ ID NO: 292 - protein, 228 aa, synthetic construct
  REGION 1..228: note = source = /note="Description of Artificial Sequence: Synthetic polypeptide"
QVQLVQSGAEVKKPGASVKVSCKASGFNIKDTYIHWVRQAPGQRLEWMGRIDPANGYTKYDPKFQGRVTITADTSASTAYMELSSLRSEDTAVYYCAREGYYGNYGVYAMDYWGQGTLVTVSSASTKGPSVFPLAPCSRSTSESTAALGCLVKDYFPEPVTVSWNSGALTSGVHTFPAVLQSSGLYSLSSVVTVPSSSLGTKTYTCNVDHKPSNTKVDKRVESKYGPP

SEQ ID NO: 293 - protein, 226 aa, synthetic construct
  REGION 1..226: note = source = /note="Description of Artificial Sequence: Synthetic polypeptide"
EVQLVESGGGLVQPGGSLRLSCAASGFTFNNYAMNWVRQAPGKGLDWVSTISGSGGTTNYADSVKGRFIISRDSSKHTLYLQMNSLRAEDTAVYYCAKDSNWGNFDLWGRGTLVTVSSASTKGPSVFPLAPSSKSTSGGTAALGCLVKDYFPEPVTVSWNSGALTSGVHTFPAVLQSSGLYSLSSVVTVPSSSLGTQTYICNVNHKPSNTKVDKKVEPKSCDKTHT

SEQ ID NO: 294 - protein, 220 aa, synthetic construct
  REGION 1..220: note = source = /note="Description of Artificial Sequence: Synthetic polypeptide"
EVQLVQSGAEVKKPGASVKVSCKASGYTLTSYGISWVRQAPGQGLEWMGWVSFYNGNTNYAQKLQGRGTMTTDPSTSTAYMELRSLRSDDTAVYYCARGYGMDVWGQGTTVTVSSASTKGPSVFPLAPCSRSTSESTAALGCLVKDYFPEPVTVSWNSGALTSGVHTFPAVLQSSGLYSLSSVVTVPSSNFGTQTYTCNVDHKPSNTKVDKTVERKCCVE

SEQ ID NO: 295 - protein, 231 aa, synthetic construct
  REGION 1..231: note = source = /note="Description of Artificial Sequence: Synthetic polypeptide"
EVQLVESGGGVIQPGGSLRLSCAASGFTFDDYAMNWVRQGPGKGLEWVSAISGDGGSTYYADSVKGRFTISRDNSKNSLYLQMNSLRAEDTAFFYCAKDLRNTIFGVVIPDAFDIWGQGTMVTVSSASTKGPSVFPLAPCSRSTSESTAALGCLVKDYFPEPVTVSWNSGALTSGVHTFPAVLQSSGLYSLSSVVTVPSSSLGTKTYTCNVDHKPSNTKVDKRVESKYGPP

SEQ ID NO: 296 - protein, 230 aa, synthetic construct
  REGION 1..230: note = source = /note="Description of Artificial Sequence: Synthetic polypeptide"
EVQLLESGGGLVQPGGSLRLSCAASGFTFSSYAMSWVRQAPGKGLEWVSGITGSGGSTYYADSVKGRFTISRDNSKNTLYLQMNSLRAEDTAVYYCAKDPGTTVIMSWFDPWGQGTLVTVSSASTKGPSVFPLAPSSKSTSGGTAALGCLVKDYFPEPVTVSWNSGALTSGVHTFPAVLQSSGLYSLSSVVTVPSSSLGTQTYICNVNHKPSNTKVDKKVEPKSCDKTHT

SEQ ID NO: 297 - protein, 218 aa, synthetic construct
  REGION 1..218: note = source = /note="Description of Artificial Sequence: Synthetic polypeptide"
QVQLVESGGGVVQPGRSLRLDCKASGITFSNSGMHWVRQAPGKGLEWVAVIWYDGSKRYYADSVKGRFTISRDNSKNTLFLQMNSLRAEDTAVYYCATNDDYWGQGTLVTVSSASTKGPSVFPLAPCSRSTSESTAALGCLVKDYFPEPVTVSWNSGALTSGVHTFPAVLQSSGLYSLSSVVTVPSSSLGTKTYTCNVDHKPSNTKVDKRVESKYGPP

SEQ ID NO: 298 - protein, 225 aa, synthetic construct
  REGION 1..225: note = source = /note="Description of Artificial Sequence: Synthetic polypeptide"
QVQLVQSGVEVKKPGASVKVSCKASGYTFTNYYMYWVRQAPGQGLEWMGGINPSNGGTNFNEKFKNRVTLTTDSSTTTAYMELKSLQFDDTAVYYCARRDYRFDMGFDYWGQGTTVTVSSASTKGPSVFPLAPCSRSTSESTAALGCLVKDYFPEPVTVSWNSGALTSGVHTFPAVLQSSGLYSLSSVVTVPSSSLGTKTYTCNVDHKPSNTKVDKRVESKYGPP

SEQ ID NO: 299 - protein, 231 aa, synthetic construct
  REGION 1..231: note = source = /note="Description of Artificial Sequence: Synthetic polypeptide"
EVQLVESGGGLVQPGGSLRLSCAASGYDFTHYGMNWVRQAPGKGLEWVGWINTYTGEPTYAADFKRRFTFSLDTSKSTAYLQMNSLRAEDTAVYYCAKYPYYYGTSHWYFDVWGQGTLVTVSSASTKGPSVFPLAPSSKSTSGGTAALGCLVKDYFPEPVTVSWNSGALTSGVHTFPAVLQSSGLYSLSSVVTVPSSSLGTQTYICNVNHKPSNTKVDKKVEPKSCDKTHL

SEQ ID NO: 300 - protein, 228 aa, synthetic construct
  REGION 1..228: note = source = /note="Description of Artificial Sequence: Synthetic polypeptide"
EVQLVESGGGLVQPGGSLRLSCSASGFTFSSFGMHWVRQAPGKGLEWVAYISSGSSTIYYGDTVKGRFTISRDNAKNSLFLQMSSLRAEDTAVYYCAREGGYYYGRSYYTMDYWGQGTTVTVSSASTKGPSVFPLAPSSKSTSGGTAALGCLVKDYFPEPVTVSWNSGALTSGVHTFPAVLQSSGLYSLSSVVTVPSSSLGTQTYICNVNHKPSNTKVDKKVEPKSCD

SEQ ID NO: 301 - protein, 231 aa, synthetic construct
  REGION 1..231: note = source = /note="Description of Artificial Sequence: Synthetic polypeptide"
EVQLVESGGGLVQPGGSLRLSCAASGYTFTNYGMNWVRQAPGKGLEWVGWINTYTGEPTYAADFKRRFTFSLDTSKSTAYLQMNSLRAEDTAVYYCAKYPHYYGSSHWYFDVWGQGTLVTVSSASTKGPSVFPLAPSSKSTSGGTAALGCLVKDYFPEPVTVSWNSGALTSGVHTFPAVLQSSGLYSLSSVVTVPSSSLGTQTYICNVNHKPSNTKVDKKVEPKSCDKTHT

SEQ ID NO: 302 - protein, 106 aa, synthetic construct
  REGION 1..106: note = source = /note="Description of Artificial Sequence: Synthetic polypeptide"
QVQLVESGGGVVQPGRSLRLSCAASGFTFSSFGMHWVRQAPGKGLEWVAVISFDGSIKYSVDSVKGRFTISRDNSKNTLFLQMNSLRAEDTAVYYCARDRLNYYDS

SEQ ID NO: 303 - protein, 220 aa, synthetic construct
  REGION 1..220: note = source = /note="Description of Artificial Sequence: Synthetic polypeptide"
EVKVVESGGGLVQPGGSMKLSCVVSGFTFSNYWVNWVRQAPGKGLEWVAQIRLKSDNYATHYEESVKGRFTISRDDSKSSVYLQMNNLRAEDSGIYYCTNWEDYWGQGTTVTVSSASTKGPSVFPLAPCSRSTSESTAALGCLVKDYFPEPVTVSWNSGALTSGVHTFPAVLQSSGLYSLSSVVTVPSSSLGTKTYTCNVDHKPSNTKVDKRVESKYGPP

SEQ ID NO: 304 - protein, 223 aa, synthetic construct
  REGION 1..223: note = source = /note="Description of Artificial Sequence: Synthetic polypeptide"
EVQLVQSGPELKKPGASVKVSCKASGYTFTNYGMNWVRQAPGQGLEWMGWINTYTGETTYADDFKGRFVFSLDTSVSTAYLQISSLKAEDTAVYYCEREGGVNNWGQGTLVTVSSASTKGPSVFPLAPSSKSTSGGTAALGCLVKDYFPEPVTVSWNSGALTSGVHTFPAVLQSSGLYSLSSVVTVPSSSLGTQTYICNVNHKPSNTKVDKKVEPKSCDKTHT

SEQ ID NO: 305 - protein, 220 aa, synthetic construct
  REGION 1..220: note = source = /note="Description of Artificial Sequence: Synthetic polypeptide"
QVQLQESGPGLVKPSETLSLTCTVSGFSLLSYGVHWVRQPPGKGLEWLGVIWTGGTTNYNSALMSRFTISKDDSKNTVYLKMNSLKTEDTAIYYCARYYYGMDYWGQGTLVTVSSASTKGPSVFPLAPCSRSTSESTAALGCLVKDYFPEPVTVSWNSGALTSGVHTFPAVLQSSGLYSLSSVVTVPSSSLGTKTYTCNVDHKPSNTKVDKRVESKYGPP

SEQ ID NO: 306 - protein, 231 aa, synthetic construct
  REGION 1..231: note = source = /note="Description of Artificial Sequence: Synthetic polypeptide"
QVQLQQSGAEVKKPGSSVRVSCKASGGTFNNNAINWVRQAPGQGLEWMGGIIPMFGTAKYSQNFQGRVAITADESTGTASMELSSLRSEDTAVYYCARSRDLLLFPHHALSPWGRGTMVTVSSASTKGPSVFPLAPSSKSTSGGTAALGCLVKDYFPEPVTVSWNSGALTSGVHTFPAVLQSSGLYSLSSVVTVPSSSLGTQTYICNVNHKPSNTKVDKKVEPKSCDKTHT

SEQ ID NO: 307 - protein, 227 aa, synthetic construct
  REGION 1..227: note = source = /note="Description of Artificial Sequence: Synthetic polypeptide"
QVQLVQSGAEVKKPGASVKVSCKASGYIFSNYWIQWVRQAPGQGLEWMGEILPGSGSTEYTENFKDRVTMTRDTSTSTVYMELSSLRSEDTAVYYCARYFFGSSPNWYFDVWGQGTLVTVSSASTKGPSVFPLAPCSRSTSESTAALGCLVKDYFPEPVTVSWNSGALTSGVHTFPAVLQSSGLYSLSSVVTVPSSNFGTQTYTCNVDHKPSNTKVDKTVERKCCVE

SEQ ID NO: 308 - protein, 230 aa, synthetic construct
  REGION 1..230: note = source = /note="Description of Artificial Sequence: Synthetic polypeptide"
EVQLLESGGGLVQPGGSLRLSCAASGFTFSHYIMMWVRQAPGKGLEWVSGIYSSGGITVYADSVKGRFTISRDNSKNTLYLQMNSLRAEDTAVYYCAYRRIGVPRRDEFDIWGQGTMVTVSSASTKGPSVFPLAPSSKSTSGGTAALGCLVKDYFPEPVTVSWNSGALTSGVHTFPAVLQSSGLYSLSSVVTVPSSSLGTQTYICNVNHKPSNTKVDKRVEPKSCDKTHT

SEQ ID NO: 309 - protein, 229 aa, synthetic construct
  REGION 1..229: note = source = /note="Description of Artificial Sequence: Synthetic polypeptide"
EVQLVESGGGLVQPGRSLRLSCAASGFTFDDYAMHWVRQAPGKGLEWVSAITWNSGHIDYADSVEGRFTISRDNAKNSLYLQMNSLRAEDTAVYYCAKVSYLSTASSLDYWGQGTLVTVSSASTKGPSVFPLAPSSKSTSGGTAALGCLVKDYFPEPVTVSWNSGALTSGVHTFPAVLQSSGLYSLSSVVTVPSSSLGTQTYICNVNHKPSNTKVDKKVEPKSCDKTHT

SEQ ID NO: 310 - protein, 228 aa, synthetic construct
  REGION 1..228: note = source = /note="Description of Artificial Sequence: Synthetic polypeptide"
EVKLEESGGGLVQPGGSMKLSCVASGFIFSNHWMNWVRQSPEKGLEWVAEIRSKSINSATHYAESVKGRFTISRDDSKSAVYLQMTDLRTEDTGVYYCSRNYYGSTYDYWGQGTTLTVSSASTKGPSVFPLAPSSKSTSGGTAALGCLVKDYFPEPVTVSWNSGALTSGVHTFPAVLQSSGLYSLSSVVTVPSSSLGTQTYICNVNHKPSNTKVDKKVEPKSCDKTHT

SEQ ID NO: 311 - protein, 55 aa, synthetic construct
  REGION 1..55: note = source = /note="Description of Artificial Sequence: Synthetic polypeptide"
QSVLTQPPSVSAAPGQKVTISCSGSSSNIGNNYVSWYQQLPGTAPKLLIYDNNKR

SEQ ID NO: 312 - protein, 110 aa, synthetic construct
  REGION 1..110: note = source = /note="Description of Artificial Sequence: Synthetic polypeptide"
EIVMTQSPSTLSASVGDRVIITCQASEIISWLAWYQQKPGKAPKLLIYLASTLASGVPSRFSGSGSGAEFTLTISSLQPDDFATYYCQNVYLASTNGANFGQGTKLTVLG

SEQ ID NO: 313 - protein, 123 aa, synthetic construct
  REGION 1..123: note = source = /note="Description of Artificial Sequence: Synthetic polypeptide"
KYYGMAVWGQGTTVTVSSASTKGPSVFPLAPCSRSTSESTAALGCLVKDYFPEPVTVSWNSGALTSGVHTFPAVLQSSGLYSLSSVVTVPSSNFGTQTYTCNVDHKPSNTKVDKTVERKCCVE

SEQ ID NO: 314 - protein, 158 aa, synthetic construct
  REGION 1..158: note = source = /note="Description of Artificial Sequence: Synthetic polypeptide"
PPDRFSGSKSGTSTTLGITGLQTGDEADYYCGTWDSRLSAVVFGGGTKLTVLGQPKANPTVTLFPPSSEELQANKATLVCLISDFYPGAVTVAWKADGSPVKAGVETTKPSKQSNNKYAASSYLSLTPEQWKSHRSYSCQVTHEGSTVEKTVAPTECS